European Patent Application EP 4 717 711 A1, published April 1, 2026. Title: ANTI-CD3 ANTIBODY AND USE THEREOF. Applicant: HEFEI TG IMMUNOPHARMA CO., LTD. The sequence listing filed with the application follows.

SEQUENCE LISTING (166 sequences)

SEQ ID NO: 1 - protein, 8 aa, synthetic construct
GFTFNTYA

SEQ ID NO: 2 - protein, 10 aa, synthetic construct
IRSKYNNYAT

SEQ ID NO: 3 - protein, 16 aa, synthetic construct
VRHGNFGNSYQSWFAY

SEQ ID NO: 4 - protein, 9 aa, synthetic construct
TGAVTTSNY

SEQ ID NO: 5 - skipped

SEQ ID NO: 6 - protein, 9 aa, synthetic construct
ALWYSNLWV

SEQ ID NO: 7 - protein, 16 aa, synthetic construct
VRHGNFGNSYVSWFLY

SEQ ID NO: 8 - protein, 16 aa, synthetic construct
VRHGNFGNSYVSWFAY

SEQ ID NO: 9 - protein, 9 aa, synthetic construct
ALWYSNDWV

SEQ ID NO: 10 - protein, 125 aa, synthetic construct
EVQLLESGGGLVQPGGSLKLSCAASGFTFNTYAMNWVRQAPGKGLEWVARIRSKYNNYATYYADSVKDRFTISRDDSKNTAYLQMNNLKTEDTAVYYCVRHGNFGNSYQSWFAYWGQGTLVTVSS

SEQ ID NO: 11 - protein, 109 aa, synthetic construct
ELVVTQEPSLTVSPGGTVTLTCRSSTGAVTTSNYANWVQQKPGQAPRGLIGGTNKRAPGTPARFSGSLLGGKAALTLSGVQPEDEAEYYCALWYSNLWVFGGGTKLTVL

SEQ ID NO: 12 - protein, 125 aa, synthetic construct
EVQLLESGGGLVQPGGSLKLSCAASGFTFNTYAMNWVRQAPGKGLEWVARIRSKYNNYATYYADSVKDRFTISRDDSKNTAYLQMNNLKTEDTAVYYCVRHGNFGNSYVSWFLYWGQGTLVTVSS

SEQ ID NO: 13 - protein, 125 aa, synthetic construct
EVQLLESGGGLVQPGGSLKLSCAASGFTFNTYAMNWVRQAPGKGLEWVARIRSKYNNYATYYADSVKDRFTISRDDSKNTAYLQMNNLKTEDTAVYYCVRHGNFGNSYVSWFAYWGQGTLVTVSS

SEQ ID NO: 14 - protein, 109 aa, synthetic construct
ELVVTQEPSLTVSPGGTVTLTCRSSTGAVTTSNYANWVQQKPGQAPRGLIGGTNKRAPGTPARFSGSLLGGKAALTLSGVQPEDEAEYYCALWYSNDWVFGGGTKLTVL

SEQ ID NO: 15 - protein, 125 aa, synthetic construct
EVQLLESGGGLVQPGGSLKLSCAASGFTFNTYAMNWVRQAPGKGLEWVARIRSKYNNYATYYADSVKDRFTISRDDSKNTAYLQMNNLKTEDTAVYYCVRHGMFGNSYVSWFAYWGQGTLVTVSS

SEQ ID NO: 16 - protein, 125 aa, synthetic construct
EVQLLESGGGLVQPGGSLKLSCAASGFTFNTYAMNWVRQAPGKGLEWVARIRSKYNNYATYYADSVKDRFTISRDDSKNTAYLQMNNLKTEDTAVYYCVRHGNFGNEYVSWFAYWGQGTLVTVSS

SEQ ID NO: 17 - protein, 125 aa, synthetic construct
EVQLLESGGGLVQPGGSLKLSCAASGFTFNTYAMNWVRQAPGKGLEWVARIRSKYNNYATYYADSVKDRFTISRDDSKNTAYLQMNNLKTEDTAVYYCVRHGNFGNPYVSWFAYWGQGTLVTVSS

SEQ ID NO: 18 - protein, 125 aa, synthetic construct
EVQLLESGGGLVQPGGSLKLSCAASGFTFNTYAMNWVRQAPGKGLEWVARIRSKYNNYATYYADSVKDRFTISRDDSKNTAYLQMNNLKTEDTAVYYCVRHGNFGNVYVSWFAYWGQGTLVTVSS

SEQ ID NO: 19 - protein, 125 aa, synthetic construct
EVQLLESGGGLVQPGGSLKLSCAASGFTFNTYAMNWVRQAPGKGLEWVARIRSKYNNYATYYADSVKDRFTISRDDSKNTAYLQMNNLKTEDTAVYYCVRHGNFGNYYVSWFAYWGQGTLVTVSS

SEQ ID NO: 20 - protein, 125 aa, synthetic construct
EVQLLESGGGLVQPGGSLKLSCAASGFTFNTYAMNWVRQAPGKGLEWVARIRSKYNNYATYYADSVKDRFTISRDDSKNTAYLQMNNLKTEDTAVYYCVRHGNFGNSEVSWFAYWGQGTLVTVSS

SEQ ID NO: 21 - protein, 125 aa, synthetic construct
EVQLLESGGGLVQPGGSLKLSCAASGFTFNTYAMNWVRQAPGKGLEWVARIRSKYNNYATYYADSVKDRFTISRDDSKNTAYLQMNNLKTEDTAVYYCVRHGNFGNSYHSWFAYWGQGTLVTVSS

SEQ ID NO: 22 - protein, 125 aa, synthetic construct
EVQLLESGGGLVQPGGSLKLSCAASGFTFNTYAMNWVRQAPGKGLEWVARIRSKYNNYATYYADSVKDRFTISRDDSKNTAYLQMNNLKTEDTAVYYCVRHGNFGNSYSSWFAYWGQGTLVTVSS

SEQ ID NO: 23 - protein, 125 aa, synthetic construct
EVQLLESGGGLVQPGGSLKLSCAASGFTFNTYAMNWVRQAPGKGLEWVARIRSKYNNYATYYADSVKDRFTISRDDSKNTAYLQMNNLKTEDTAVYYCVRHGNFGNSYVSWFAGWGQGTLVTVSS

SEQ ID NO: 24 - protein, 125 aa, synthetic construct
EVQLLESGGGLVQPGGSLKLSCAASGFTFNTYAMNWVRQAPGKGLEWVARIRSKYNNYATYYADSVKDRFTISRDDSKNTAYLQMNNLKTEDTAVYYCVRHGNFGNSYVSWFAMWGQGTLVTVSS

SEQ ID NO: 25 - protein, 109 aa, synthetic construct
ELVVTQEPSLTVSPGGTVTLTCRSSTGAVTTSNYANWVQQKPGQAPRGLIGGTNKRAPGTPARFSGSLLGGKAALTLSGVQPEDEAEYYCALWYPNLWVFGGGTKLTVL

SEQ ID NO: 26 - protein, 109 aa, synthetic construct
ELVVTQEPSLTVSPGGTVTLTCRSSTGAVTTSNYANWVQQKPGQAPRGLIGGTNKRAPGTPARFSGSLLGGKAALTLSGVQPEDEAEYYCALWYSNPWVFGGGTKLTVL

SEQ ID NO: 27 - protein, 125 aa, synthetic construct; identical to SEQ ID NO: 15

SEQ ID NO: 28 - protein, 109 aa, synthetic construct
ELVVTQEPSLTVSPGGTVTLTCRSSTGAVTTSNYANWVQQKPGQAPRGLIGGTNKRAPGTPARFSGSLLGGKAALTLSGVQPEDEAEYYCALWYPNPWVFGGGTKLTVL

SEQ ID NO: 29 - protein, 125 aa, synthetic construct; identical to SEQ ID NO: 12

SEQ ID NO: 30 - protein, 109 aa, synthetic construct
ELVVTQEPSLTVSPGGTVTLTCRSSTGAVTTSNYANWVQQKPGQAPRGLIGGTNKRAPGTPARFSGSLLGGKAALTLSGVQPEDEAEYYCALWYPNDWVFGGGTKLTVL

SEQ ID NO: 31 - protein, 125 aa, synthetic construct
EVQLLESGGGLVQPGGSLKLSCAASGFTFNTYAMNWVRQAPGKGLEWVARIRSKYNNYATYYADSVKDRFTISRDDSKNTAYLQMNNLKTEDTAVYYCVRHGNFGNDYVSWFAYWGQGTLVTVSS

SEQ ID NO: 32 - protein, 455 aa, synthetic construct
EVQLLESGGGLVQPGGSLKLSCAASGFTFNTYAMNWVRQAPGKGLEWVARIRSKYNNYATYYADSVKDRFTISRDDSKNTAYLQMNNLKTEDTAVYYCVRHGNFGNSYQSWFAYWGQGTLVTVSSASTKGPSVFPLAPSSKSTSGGTAALGCLVKDYFPEPVTVSWNSGALTSGVHTFPAVLQSSGLYSLSSVVTVPSSSLGTQTYICNVNHKPSNTKVDKKVEPKSCDKTHTCPPCPAPELLGGPSVFLFPPKPKDTLMISRTPEVTCVVVDVSHEDPEVKFNWYVDGVEVHNAKTKPREEQYNSTYRVVSVLTVLHQDWLNGKEYKCKVSNKALPAPIEKTISKAKGQPREPQVYTLPPSREEMTKNQVSLTCLVKGFYPSDIAVEWESNGQPENNYKTTPPVLDSDGSFFLYSKLTVDKSRWQQGNVFSCSVMHEALHNHYTQKSLSLSPGK

SEQ ID NO: 33 - protein, 216 aa, synthetic construct
ELVVTQEPSLTVSPGGTVTLTCRSSTGAVTTSNYANWVQQKPGQAPRGLIGGTNKRAPGTPARFSGSLLGGKAALTLSGVQPEDEAEYYCALWYSNLWVFGGGTKLTVLRTVAAPSVFIFPPSDEQLKSGTASVVCLLNNFYPREAKVQWKVDNALQSGNSQESVTEQDSKDSTYSLSSTLTLSKADYEKHKVYACEVTHQGLSSPVTKSFNRGEC

SEQ ID NO: 34 - protein, 455 aa, synthetic construct
EVQLLESGGGLVQPGGSLKLSCAASGFTFNTYAMNWVRQAPGKGLEWVARIRSKYNNYATYYADSVKDRFTISRDDSKNTAYLQMNNLKTEDTAVYYCVRHGNFGNSYVSWFLYWGQGTLVTVSSASTKGPSVFPLAPSSKSTSGGTAALGCLVKDYFPEPVTVSWNSGALTSGVHTFPAVLQSSGLYSLSSVVTVPSSSLGTQTYICNVNHKPSNTKVDKKVEPKSCDKTHTCPPCPAPELLGGPSVFLFPPKPKDTLMISRTPEVTCVVVDVSHEDPEVKFNWYVDGVEVHNAKTKPREEQYNSTYRVVSVLTVLHQDWLNGKEYKCKVSNKALPAPIEKTISKAKGQPREPQVYTLPPSREEMTKNQVSLTCLVKGFYPSDIAVEWESNGQPENNYKTTPPVLDSDGSFFLYSKLTVDKSRWQQGNVFSCSVMHEALHNHYTQKSLSLSPGK

SEQ ID NO: 35 - protein, 455 aa, synthetic construct
EVQLLESGGGLVQPGGSLKLSCAASGFTFNTYAMNWVRQAPGKGLEWVARIRSKYNNYATYYADSVKDRFTISRDDSKNTAYLQMNNLKTEDTAVYYCVRHGNFGNSYVSWFAYWGQGTLVTVSSASTKGPSVFPLAPSSKSTSGGTAALGCLVKDYFPEPVTVSWNSGALTSGVHTFPAVLQSSGLYSLSSVVTVPSSSLGTQTYICNVNHKPSNTKVDKKVEPKSCDKTHTCPPCPAPELLGGPSVFLFPPKPKDTLMISRTPEVTCVVVDVSHEDPEVKFNWYVDGVEVHNAKTKPREEQYNSTYRVVSVLTVLHQDWLNGKEYKCKVSNKALPAPIEKTISKAKGQPREPQVYTLPPSREEMTKNQVSLTCLVKGFYPSDIAVEWESNGQPENNYKTTPPVLDSDGSFFLYSKLTVDKSRWQQGNVFSCSVMHEALHNHYTQKSLSLSPGK

SEQ ID NO: 36 - protein, 216 aa, synthetic construct
ELVVTQEPSLTVSPGGTVTLTCRSSTGAVTTSNYANWVQQKPGQAPRGLIGGTNKRAPGTPARFSGSLLGGKAALTLSGVQPEDEAEYYCALWYSNDWVFGGGTKLTVLRTVAAPSVFIFPPSDEQLKSGTASVVCLLNNFYPREAKVQWKVDNALQSGNSQESVTEQDSKDSTYSLSSTLTLSKADYEKHKVYACEVTHQGLSSPVTKSFNRGEC

SEQ ID NO: 37 - protein, 455 aa, synthetic construct
EVQLLESGGGLVQPGGSLKLSCAASGFTFNTYAMNWVRQAPGKGLEWVARIRSKYNNYATYYADSVKDRFTISRDDSKNTAYLQMNNLKTEDTAVYYCVRHGMFGNSYVSWFAYWGQGTLVTVSSASTKGPSVFPLAPSSKSTSGGTAALGCLVKDYFPEPVTVSWNSGALTSGVHTFPAVLQSSGLYSLSSVVTVPSSSLGTQTYICNVNHKPSNTKVDKKVEPKSCDKTHTCPPCPAPELLGGPSVFLFPPKPKDTLMISRTPEVTCVVVDVSHEDPEVKFNWYVDGVEVHNAKTKPREEQYNSTYRVVSVLTVLHQDWLNGKEYKCKVSNKALPAPIEKTISKAKGQPREPQVYTLPPSREEMTKNQVSLTCLVKGFYPSDIAVEWESNGQPENNYKTTPPVLDSDGSFFLYSKLTVDKSRWQQGNVFSCSVMHEALHNHYTQKSLSLSPGK

SEQ ID NO: 38 - protein, 455 aa, synthetic construct
EVQLLESGGGLVQPGGSLKLSCAASGFTFNTYAMNWVRQAPGKGLEWVARIRSKYNNYATYYADSVKDRFTISRDDSKNTAYLQMNNLKTEDTAVYYCVRHGNFGNEYVSWFAYWGQGTLVTVSSASTKGPSVFPLAPSSKSTSGGTAALGCLVKDYFPEPVTVSWNSGALTSGVHTFPAVLQSSGLYSLSSVVTVPSSSLGTQTYICNVNHKPSNTKVDKKVEPKSCDKTHTCPPCPAPELLGGPSVFLFPPKPKDTLMISRTPEVTCVVVDVSHEDPEVKFNWYVDGVEVHNAKTKPREEQYNSTYRVVSVLTVLHQDWLNGKEYKCKVSNKALPAPIEKTISKAKGQPREPQVYTLPPSREEMTKNQVSLTCLVKGFYPSDIAVEWESNGQPENNYKTTPPVLDSDGSFFLYSKLTVDKSRWQQGNVFSCSVMHEALHNHYTQKSLSLSPGK

SEQ ID NO: 39 - protein, 455 aa, synthetic construct
EVQLLESGGGLVQPGGSLKLSCAASGFTFNTYAMNWVRQAPGKGLEWVARIRSKYNNYATYYADSVKDRFTISRDDSKNTAYLQMNNLKTEDTAVYYCVRHGNFGNPYVSWFAYWGQGTLVTVSSASTKGPSVFPLAPSSKSTSGGTAALGCLVKDYFPEPVTVSWNSGALTSGVHTFPAVLQSSGLYSLSSVVTVPSSSLGTQTYICNVNHKPSNTKVDKKVEPKSCDKTHTCPPCPAPELLGGPSVFLFPPKPKDTLMISRTPEVTCVVVDVSHEDPEVKFNWYVDGVEVHNAKTKPREEQYNSTYRVVSVLTVLHQDWLNGKEYKCKVSNKALPAPIEKTISKAKGQPREPQVYTLPPSREEMTKNQVSLTCLVKGFYPSDIAVEWESNGQPENNYKTTPPVLDSDGSFFLYSKLTVDKSRWQQGNVFSCSVMHEALHNHYTQKSLSLSPGK

SEQ ID NO: 40 - protein, 455 aa, synthetic construct
EVQLLESGGGLVQPGGSLKLSCAASGFTFNTYAMNWVRQAPGKGLEWVARIRSKYNNYATYYADSVKDRFTISRDDSKNTAYLQMNNLKTEDTAVYYCVRHGNFGNVYVSWFAYWGQGTLVTVSSASTKGPSVFPLAPSSKSTSGGTAALGCLVKDYFPEPVTVSWNSGALTSGVHTFPAVLQSSGLYSLSSVVTVPSSSLGTQTYICNVNHKPSNTKVDKKVEPKSCDKTHTCPPCPAPELLGGPSVFLFPPKPKDTLMISRTPEVTCVVVDVSHEDPEVKFNWYVDGVEVHNAKTKPREEQYNSTYRVVSVLTVLHQDWLNGKEYKCKVSNKALPAPIEKTISKAKGQPREPQVYTLPPSREEMTKNQVSLTCLVKGFYPSDIAVEWESNGQPENNYKTTPPVLDSDGSFFLYSKLTVDKSRWQQGNVFSCSVMHEALHNHYTQKSLSLSPGK

SEQ ID NO: 41 - protein, 455 aa, synthetic construct
EVQLLESGGGLVQPGGSLKLSCAASGFTFNTYAMNWVRQAPGKGLEWVARIRSKYNNYATYYADSVKDRFTISRDDSKNTAYLQMNNLKTEDTAVYYCVRHGNFGNYYVSWFAYWGQGTLVTVSSASTKGPSVFPLAPSSKSTSGGTAALGCLVKDYFPEPVTVSWNSGALTSGVHTFPAVLQSSGLYSLSSVVTVPSSSLGTQTYICNVNHKPSNTKVDKKVEPKSCDKTHTCPPCPAPELLGGPSVFLFPPKPKDTLMISRTPEVTCVVVDVSHEDPEVKFNWYVDGVEVHNAKTKPREEQYNSTYRVVSVLTVLHQDWLNGKEYKCKVSNKALPAPIEKTISKAKGQPREPQVYTLPPSREEMTKNQVSLTCLVKGFYPSDIAVEWESNGQPENNYKTTPPVLDSDGSFFLYSKLTVDKSRWQQGNVFSCSVMHEALHNHYTQKSLSLSPGK

SEQ ID NO: 42 - protein, 455 aa, synthetic construct
EVQLLESGGGLVQPGGSLKLSCAASGFTFNTYAMNWVRQAPGKGLEWVARIRSKYNNYATYYADSVKDRFTISRDDSKNTAYLQMNNLKTEDTAVYYCVRHGNFGNSEVSWFAYWGQGTLVTVSSASTKGPSVFPLAPSSKSTSGGTAALGCLVKDYFPEPVTVSWNSGALTSGVHTFPAVLQSSGLYSLSSVVTVPSSSLGTQTYICNVNHKPSNTKVDKKVEPKSCDKTHTCPPCPAPELLGGPSVFLFPPKPKDTLMISRTPEVTCVVVDVSHEDPEVKFNWYVDGVEVHNAKTKPREEQYNSTYRVVSVLTVLHQDWLNGKEYKCKVSNKALPAPIEKTISKAKGQPREPQVYTLPPSREEMTKNQVSLTCLVKGFYPSDIAVEWESNGQPENNYKTTPPVLDSDGSFFLYSKLTVDKSRWQQGNVFSCSVMHEALHNHYTQKSLSLSPGK

SEQ ID NO: 43 - protein, 455 aa, synthetic construct
EVQLLESGGGLVQPGGSLKLSCAASGFTFNTYAMNWVRQAPGKGLEWVARIRSKYNNYATYYADSVKDRFTISRDDSKNTAYLQMNNLKTEDTAVYYCVRHGNFGNSYHSWFAYWGQGTLVTVSSASTKGPSVFPLAPSSKSTSGGTAALGCLVKDYFPEPVTVSWNSGALTSGVHTFPAVLQSSGLYSLSSVVTVPSSSLGTQTYICNVNHKPSNTKVDKKVEPKSCDKTHTCPPCPAPELLGGPSVFLFPPKPKDTLMISRTPEVTCVVVDVSHEDPEVKFNWYVDGVEVHNAKTKPREEQYNSTYRVVSVLTVLHQDWLNGKEYKCKVSNKALPAPIEKTISKAKGQPREPQVYTLPPSREEMTKNQVSLTCLVKGFYPSDIAVEWESNGQPENNYKTTPPVLDSDGSFFLYSKLTVDKSRWQQGNVFSCSVMHEALHNHYTQKSLSLSPGK

SEQ ID NO: 44 - protein, 455 aa, synthetic construct
EVQLLESGGGLVQPGGSLKLSCAASGFTFNTYAMNWVRQAPGKGLEWVARIRSKYNNYATYYADSVKDRFTISRDDSKNTAYLQMNNLKTEDTAVYYCVRHGNFGNSYSSWFAYWGQGTLVTVSSASTKGPSVFPLAPSSKSTSGGTAALGCLVKDYFPEPVTVSWNSGALTSGVHTFPAVLQSSGLYSLSSVVTVPSSSLGTQTYICNVNHKPSNTKVDKKVEPKSCDKTHTCPPCPAPELLGGPSVFLFPPKPKDTLMISRTPEVTCVVVDVSHEDPEVKFNWYVDGVEVHNAKTKPREEQYNSTYRVVSVLTVLHQDWLNGKEYKCKVSNKALPAPIEKTISKAKGQPREPQVYTLPPSREEMTKNQVSLTCLVKGFYPSDIAVEWESNGQPENNYKTTPPVLDSDGSFFLYSKLTVDKSRWQQGNVFSCSVMHEALHNHYTQKSLSLSPGK

SEQ ID NO: 45 - protein, 455 aa, synthetic construct
EVQLLESGGGLVQPGGSLKLSCAASGFTFNTYAMNWVRQAPGKGLEWVARIRSKYNNYATYYADSVKDRFTISRDDSKNTAYLQMNNLKTEDTAVYYCVRHGNFGNSYVSWFAGWGQGTLVTVSSASTKGPSVFPLAPSSKSTSGGTAALGCLVKDYFPEPVTVSWNSGALTSGVHTFPAVLQSSGLYSLSSVVTVPSSSLGTQTYICNVNHKPSNTKVDKKVEPKSCDKTHTCPPCPAPELLGGPSVFLFPPKPKDTLMISRTPEVTCVVVDVSHEDPEVKFNWYVDGVEVHNAKTKPREEQYNSTYRVVSVLTVLHQDWLNGKEYKCKVSNKALPAPIEKTISKAKGQPREPQVYTLPPSREEMTKNQVSLTCLVKGFYPSDIAVEWESNGQPENNYKTTPPVLDSDGSFFLYSKLTVDKSRWQQGNVFSCSVMHEALHNHYTQKSLSLSPGK

SEQ ID NO: 46 - protein, 455 aa, synthetic construct
EVQLLESGGGLVQPGGSLKLSCAASGFTFNTYAMNWVRQAPGKGLEWVARIRSKYNNYATYYADSVKDRFTISRDDSKNTAYLQMNNLKTEDTAVYYCVRHGNFGNSYVSWFAMWGQGTLVTVSSASTKGPSVFPLAPSSKSTSGGTAALGCLVKDYFPEPVTVSWNSGALTSGVHTFPAVLQSSGLYSLSSVVTVPSSSLGTQTYICNVNHKPSNTKVDKKVEPKSCDKTHTCPPCPAPELLGGPSVFLFPPKPKDTLMISRTPEVTCVVVDVSHEDPEVKFNWYVDGVEVHNAKTKPREEQYNSTYRVVSVLTVLHQDWLNGKEYKCKVSNKALPAPIEKTISKAKGQPREPQVYTLPPSREEMTKNQVSLTCLVKGFYPSDIAVEWESNGQPENNYKTTPPVLDSDGSFFLYSKLTVDKSRWQQGNVFSCSVMHEALHNHYTQKSLSLSPGK

SEQ ID NO: 47 - protein, 216 aa, synthetic construct
ELVVTQEPSLTVSPGGTVTLTCRSSTGAVTTSNYANWVQQKPGQAPRGLIGGTNKRAPGTPARFSGSLLGGKAALTLSGVQPEDEAEYYCALWYPNLWVFGGGTKLTVLRTVAAPSVFIFPPSDEQLKSGTASVVCLLNNFYPREAKVQWKVDNALQSGNSQESVTEQDSKDSTYSLSSTLTLSKADYEKHKVYACEVTHQGLSSPVTKSFNRGEC

SEQ ID NO: 48 - protein, 216 aa, synthetic construct
ELVVTQEPSLTVSPGGTVTLTCRSSTGAVTTSNYANWVQQKPGQAPRGLIGGTNKRAPGTPARFSGSLLGGKAALTLSGVQPEDEAEYYCALWYSNPWVFGGGTKLTVLRTVAAPSVFIFPPSDEQLKSGTASVVCLLNNFYPREAKVQWKVDNALQSGNSQESVTEQDSKDSTYSLSSTLTLSKADYEKHKVYACEVTHQGLSSPVTKSFNRGEC

SEQ ID NO: 49 - protein, 485 aa, synthetic construct
EVQLLESGGGLVQPGGSLKLSCAASGFTFNTYAMNWVRQAPGKGLEWVARIRSKYNNYATYYADSVKDRFTISRDDSKNTAYLQMNNLKTEDTAVYYCVRHGNFGNSYQSWFAYWGQGTLVTVSSGGGGSGGGGSGGGGSELVVTQEPSLTVSPGGTVTLTCRSSTGAVTTSNYANWVQQKPGQAPRGLIGGTNKRAPGTPARFSGSLLGGKAALTLSGVQPEDEAEYYCALWYSNLWVFGGGTKLTVLGGGGSPKSSDKTHTCPPCPAPEAAGGPSVFLFPPKPKDTLMISRTPEVTCVVVDVSHEDPEVKFNWYVDGVEVHNAKTKPREEQYNSTYRVVSVLTVLHQDWLNGKEYKCKVSNKALPAPIEKTISKAKGQPREPQVYTLPPCREEMTKNQVSLWCLVKGFYPSDIAVEWESNGQPENNYKTTPPVLDSDGSFFLYSKLTVDKSRWQQGNVFSCSVMHEALHNHYTQKSLSLSPGK

SEQ ID NO: 50 - protein, 485 aa, synthetic construct
EVQLLESGGGLVQPGGSLKLSCAASGFTFNTYAMNWVRQAPGKGLEWVARIRSKYNNYATYYADSVKDRFTISRDDSKNTAYLQMNNLKTEDTAVYYCVRHGNFGNSYVSWFLYWGQGTLVTVSSGGGGSGGGGSGGGGSELVVTQEPSLTVSPGGTVTLTCRSSTGAVTTSNYANWVQQKPGQAPRGLIGGTNKRAPGTPARFSGSLLGGKAALTLSGVQPEDEAEYYCALWYSNLWVFGGGTKLTVLGGGGSPKSSDKTHTCPPCPAPEAAGGPSVFLFPPKPKDTLMISRTPEVTCVVVDVSHEDPEVKFNWYVDGVEVHNAKTKPREEQYNSTYRVVSVLTVLHQDWLNGKEYKCKVSNKALPAPIEKTISKAKGQPREPQVYTLPPCREEMTKNQVSLWCLVKGFYPSDIAVEWESNGQPENNYKTTPPVLDSDGSFFLYSKLTVDKSRWQQGNVFSCSVMHEALHNHYTQKSLSLSPGK

SEQ ID NO: 51 - protein, 485 aa, synthetic construct
EVQLLESGGGLVQPGGSLKLSCAASGFTFNTYAMNWVRQAPGKGLEWVARIRSKYNNYATYYADSVKDRFTISRDDSKNTAYLQMNNLKTEDTAVYYCVRHGNFGNSYVSWFAYWGQGTLVTVSSGGGGSGGGGSGGGGSELVVTQEPSLTVSPGGTVTLTCRSSTGAVTTSNYANWVQQKPGQAPRGLIGGTNKRAPGTPARFSGSLLGGKAALTLSGVQPEDEAEYYCALWYSNDWVFGGGTKLTVLGGGGSPKSSDKTHTCPPCPAPEAAGGPSVFLFPPKPKDTLMISRTPEVTCVVVDVSHEDPEVKFNWYVDGVEVHNAKTKPREEQYNSTYRVVSVLTVLHQDWLNGKEYKCKVSNKALPAPIEKTISKAKGQPREPQVYTLPPCREEMTKNQVSLWCLVKGFYPSDIAVEWESNGQPENNYKTTPPVLDSDGSFFLYSKLTVDKSRWQQGNVFSCSVMHEALHNHYTQKSLSLSPGK

SEQ ID NO: 52 - protein, 485 aa, synthetic construct
EVQLLESGGGLVQPGGSLKLSCAASGFTFNTYAMNWVRQAPGKGLEWVARIRSKYNNYATYYADSVKDRFTISRDDSKNTAYLQMNNLKTEDTAVYYCVRHGNFGNSYVSWFAYWGQGTLVTVSSGGGGSGGGGSGGGGSELVVTQEPSLTVSPGGTVTLTCRSSTGAVTTSNYANWVQQKPGQAPRGLIGGTNKRAPGTPARFSGSLLGGKAALTLSGVQPEDEAEYYCALWYSNLWVFGGGTKLTVLGGGGSPKSSDKTHTCPPCPAPEAAGGPSVFLFPPKPKDTLMISRTPEVTCVVVDVSHEDPEVKFNWYVDGVEVHNAKTKPREEQYNSTYRVVSVLTVLHQDWLNGKEYKCKVSNKALPAPIEKTISKAKGQPREPQVYTLPPCREEMTKNQVSLWCLVKGFYPSDIAVEWESNGQPENNYKTTPPVLDSDGSFFLYSKLTVDKSRWQQGNVFSCSVMHEALHNHYTQKSLSLSPGK

SEQ ID NO: 53 - protein, 485 aa, synthetic construct
EVQLLESGGGLVQPGGSLKLSCAASGFTFNTYAMNWVRQAPGKGLEWVARIRSKYNNYATYYADSVKDRFTISRDDSKNTAYLQMNNLKTEDTAVYYCVRHGMFGNSYVSWFAYWGQGTLVTVSSGGGGSGGGGSGGGGSELVVTQEPSLTVSPGGTVTLTCRSSTGAVTTSNYANWVQQKPGQAPRGLIGGTNKRAPGTPARFSGSLLGGKAALTLSGVQPEDEAEYYCALWYSNLWVFGGGTKLTVLGGGGSPKSSDKTHTCPPCPAPEAAGGPSVFLFPPKPKDTLMISRTPEVTCVVVDVSHEDPEVKFNWYVDGVEVHNAKTKPREEQYNSTYRVVSVLTVLHQDWLNGKEYKCKVSNKALPAPIEKTISKAKGQPREPQVYTLPPCREEMTKNQVSLWCLVKGFYPSDIAVEWESNGQPENNYKTTPPVLDSDGSFFLYSKLTVDKSRWQQGNVFSCSVMHEALHNHYTQKSLSLSPGK

SEQ ID NO: 54 - protein, 485 aa, synthetic construct
EVQLLESGGGLVQPGGSLKLSCAASGFTFNTYAMNWVRQAPGKGLEWVARIRSKYNNYATYYADSVKDRFTISRDDSKNTAYLQMNNLKTEDTAVYYCVRHGNFGNEYVSWFAYWGQGTLVTVSSGGGGSGGGGSGGGGSELVVTQEPSLTVSPGGTVTLTCRSSTGAVTTSNYANWVQQKPGQAPRGLIGGTNKRAPGTPARFSGSLLGGKAALTLSGVQPEDEAEYYCALWYSNLWVFGGGTKLTVLGGGGSPKSSDKTHTCPPCPAPEAAGGPSVFLFPPKPKDTLMISRTPEVTCVVVDVSHEDPEVKFNWYVDGVEVHNAKTKPREEQYNSTYRVVSVLTVLHQDWLNGKEYKCKVSNKALPAPIEKTISKAKGQPREPQVYTLPPCREEMTKNQVSLWCLVKGFYPSDIAVEWESNGQPENNYKTTPPVLDSDGSFFLYSKLTVDKSRWQQGNVFSCSVMHEALHNHYTQKSLSLSPGK

SEQ ID NO: 55 - protein, 485 aa, synthetic construct
EVQLLESGGGLVQPGGSLKLSCAASGFTFNTYAMNWVRQAPGKGLEWVARIRSKYNNYATYYADSVKDRFTISRDDSKNTAYLQMNNLKTEDTAVYYCVRHGNFGNPYVSWFAYWGQGTLVTVSSGGGGSGGGGSGGGGSELVVTQEPSLTVSPGGTVTLTCRSSTGAVTTSNYANWVQQKPGQAPRGLIGGTNKRAPGTPARFSGSLLGGKAALTLSGVQPEDEAEYYCALWYSNLWVFGGGTKLTVLGGGGSPKSSDKTHTCPPCPAPEAAGGPSVFLFPPKPKDTLMISRTPEVTCVVVDVSHEDPEVKFNWYVDGVEVHNAKTKPREEQYNSTYRVVSVLTVLHQDWLNGKEYKCKVSNKALPAPIEKTISKAKGQPREPQVYTLPPCREEMTKNQVSLWCLVKGFYPSDIAVEWESNGQPENNYKTTPPVLDSDGSFFLYSKLTVDKSRWQQGNVFSCSVMHEALHNHYTQKSLSLSPGK

SEQ ID NO: 56 - protein, 485 aa, synthetic construct
EVQLLESGGGLVQPGGSLKLSCAASGFTFNTYAMNWVRQAPGKGLEWVARIRSKYNNYATYYADSVKDRFTISRDDSKNTAYLQMNNLKTEDTAVYYCVRHGNFGNVYVSWFAYWGQGTLVTVSSGGGGSGGGGSGGGGSELVVTQEPSLTVSPGGTVTLTCRSSTGAVTTSNYANWVQQKPGQAPRGLIGGTNKRAPGTPARFSGSLLGGKAALTLSGVQPEDEAEYYCALWYSNLWVFGGGTKLTVLGGGGSPKSSDKTHTCPPCPAPEAAGGPSVFLFPPKPKDTLMISRTPEVTCVVVDVSHEDPEVKFNWYVDGVEVHNAKTKPREEQYNSTYRVVSVLTVLHQDWLNGKEYKCKVSNKALPAPIEKTISKAKGQPREPQVYTLPPCREEMTKNQVSLWCLVKGFYPSDIAVEWESNGQPENNYKTTPPVLDSDGSFFLYSKLTVDKSRWQQGNVFSCSVMHEALHNHYTQKSLSLSPGK

SEQ ID NO: 57 - protein, 485 aa, synthetic construct
EVQLLESGGGLVQPGGSLKLSCAASGFTFNTYAMNWVRQAPGKGLEWVARIRSKYNNYATYYADSVKDRFTISRDDSKNTAYLQMNNLKTEDTAVYYCVRHGNFGNYYVSWFAYWGQGTLVTVSSGGGGSGGGGSGGGGSELVVTQEPSLTVSPGGTVTLTCRSSTGAVTTSNYANWVQQKPGQAPRGLIGGTNKRAPGTPARFSGSLLGGKAALTLSGVQPEDEAEYYCALWYSNLWVFGGGTKLTVLGGGGSPKSSDKTHTCPPCPAPEAAGGPSVFLFPPKPKDTLMISRTPEVTCVVVDVSHEDPEVKFNWYVDGVEVHNAKTKPREEQYNSTYRVVSVLTVLHQDWLNGKEYKCKVSNKALPAPIEKTISKAKGQPREPQVYTLPPCREEMTKNQVSLWCLVKGFYPSDIAVEWESNGQPENNYKTTPPVLDSDGSFFLYSKLTVDKSRWQQGNVFSCSVMHEALHNHYTQKSLSLSPGK

SEQ ID NO: 58 - protein, 485 aa, synthetic construct
EVQLLESGGGLVQPGGSLKLSCAASGFTFNTYAMNWVRQAPGKGLEWVARIRSKYNNYATYYADSVKDRFTISRDDSKNTAYLQMNNLKTEDTAVYYCVRHGNFGNSEVSWFAYWGQGTLVTVSSGGGGSGGGGSGGGGSELVVTQEPSLTVSPGGTVTLTCRSSTGAVTTSNYANWVQQKPGQAPRGLIGGTNKRAPGTPARFSGSLLGGKAALTLSGVQPEDEAEYYCALWYSNLWVFGGGTKLTVLGGGGSPKSSDKTHTCPPCPAPEAAGGPSVFLFPPKPKDTLMISRTPEVTCVVVDVSHEDPEVKFNWYVDGVEVHNAKTKPREEQYNSTYRVVSVLTVLHQDWLNGKEYKCKVSNKALPAPIEKTISKAKGQPREPQVYTLPPCREEMTKNQVSLWCLVKGFYPSDIAVEWESNGQPENNYKTTPPVLDSDGSFFLYSKLTVDKSRWQQGNVFSCSVMHEALHNHYTQKSLSLSPGK

SEQ ID NO: 59 - protein, 485 aa, synthetic construct
EVQLLESGGGLVQPGGSLKLSCAASGFTFNTYAMNWVRQAPGKGLEWVARIRSKYNNYATYYADSVKDRFTISRDDSKNTAYLQMNNLKTEDTAVYYCVRHGNFGNSYHSWFAYWGQGTLVTVSSGGGGSGGGGSGGGGSELVVTQEPSLTVSPGGTVTLTCRSSTGAVTTSNYANWVQQKPGQAPRGLIGGTNKRAPGTPARFSGSLLGGKAALTLSGVQPEDEAEYYCALWYSNLWVFGGGTKLTVLGGGGSPKSSDKTHTCPPCPAPEAAGGPSVFLFPPKPKDTLMISRTPEVTCVVVDVSHEDPEVKFNWYVDGVEVHNAKTKPREEQYNSTYRVVSVLTVLHQDWLNGKEYKCKVSNKALPAPIEKTISKAKGQPREPQVYTLPPCREEMTKNQVSLWCLVKGFYPSDIAVEWESNGQPENNYKTTPPVLDSDGSFFLYSKLTVDKSRWQQGNVFSCSVMHEALHNHYTQKSLSLSPGK

SEQ ID NO: 60 - protein, 485 aa, synthetic construct
EVQLLESGGGLVQPGGSLKLSCAASGFTFNTYAMNWVRQAPGKGLEWVARIRSKYNNYATYYADSVKDRFTISRDDSKNTAYLQMNNLKTEDTAVYYCVRHGNFGNSYSSWFAYWGQGTLVTVSSGGGGSGGGGSGGGGSELVVTQEPSLTVSPGGTVTLTCRSSTGAVTTSNYANWVQQKPGQAPRGLIGGTNKRAPGTPARFSGSLLGGKAALTLSGVQPEDEAEYYCALWYSNLWVFGGGTKLTVLGGGGSPKSSDKTHTCPPCPAPEAAGGPSVFLFPPKPKDTLMISRTPEVTCVVVDVSHEDPEVKFNWYVDGVEVHNAKTKPREEQYNSTYRVVSVLTVLHQDWLNGKEYKCKVSNKALPAPIEKTISKAKGQPREPQVYTLPPCREEMTKNQVSLWCLVKGFYPSDIAVEWESNGQPENNYKTTPPVLDSDGSFFLYSKLTVDKSRWQQGNVFSCSVMHEALHNHYTQKSLSLSPGK

SEQ ID NO: 61 - protein, 485 aa, synthetic construct
EVQLLESGGGLVQPGGSLKLSCAASGFTFNTYAMNWVRQAPGKGLEWVARIRSKYNNYATYYADSVKDRFTISRDDSKNTAYLQMNNLKTEDTAVYYCVRHGNFGNSYVSWFAGWGQGTLVTVSSGGGGSGGGGSGGGGSELVVTQEPSLTVSPGGTVTLTCRSSTGAVTTSNYANWVQQKPGQAPRGLIGGTNKRAPGTPARFSGSLLGGKAALTLSGVQPEDEAEYYCALWYSNLWVFGGGTKLTVLGGGGSPKSSDKTHTCPPCPAPEAAGGPSVFLFPPKPKDTLMISRTPEVTCVVVDVSHEDPEVKFNWYVDGVEVHNAKTKPREEQYNSTYRVVSVLTVLHQDWLNGKEYKCKVSNKALPAPIEKTISKAKGQPREPQVYTLPPCREEMTKNQVSLWCLVKGFYPSDIAVEWESNGQPENNYKTTPPVLDSDGSFFLYSKLTVDKSRWQQGNVFSCSVMHEALHNHYTQKSLSLSPGK

SEQ ID NO: 62 - protein, 485 aa, synthetic construct
EVQLLESGGGLVQPGGSLKLSCAASGFTFNTYAMNWVRQAPGKGLEWVARIRSKYNNYATYYADSVKDRFTISRDDSKNTAYLQMNNLKTEDTAVYYCVRHGNFGNSYVSWFAMWGQGTLVTVSSGGGGSGGGGSGGGGSELVVTQEPSLTVSPGGTVTLTCRSSTGAVTTSNYANWVQQKPGQAPRGLIGGTNKRAPGTPARFSGSLLGGKAALTLSGVQPEDEAEYYCALWYSNLWVFGGGTKLTVLGGGGSPKSSDKTHTCPPCPAPEAAGGPSVFLFPPKPKDTLMISRTPEVTCVVVDVSHEDPEVKFNWYVDGVEVHNAKTKPREEQYNSTYRVVSVLTVLHQDWLNGKEYKCKVSNKALPAPIEKTISKAKGQPREPQVYTLPPCREEMTKNQVSLWCLVKGFYPSDIAVEWESNGQPENNYKTTPPVLDSDGSFFLYSKLTVDKSRWQQGNVFSCSVMHEALHNHYTQKSLSLSPGK

SEQ ID NO: 63 - protein, 485 aa, synthetic construct
EVQLLESGGGLVQPGGSLKLSCAASGFTFNTYAMNWVRQAPGKGLEWVARIRSKYNNYATYYADSVKDRFTISRDDSKNTAYLQMNNLKTEDTAVYYCVRHGNFGNSYVSWFAYWGQGTLVTVSSGGGGSGGGGSGGGGSELVVTQEPSLTVSPGGTVTLTCRSSTGAVTTSNYANWVQQKPGQAPRGLIGGTNKRAPGTPARFSGSLLGGKAALTLSGVQPEDEAEYYCALWYPNLWVFGGGTKLTVLGGGGSPKSSDKTHTCPPCPAPEAAGGPSVFLFPPKPKDTLMISRTPEVTCVVVDVSHEDPEVKFNWYVDGVEVHNAKTKPREEQYNSTYRVVSVLTVLHQDWLNGKEYKCKVSNKALPAPIEKTISKAKGQPREPQVYTLPPCREEMTKNQVSLWCLVKGFYPSDIAVEWESNGQPENNYKTTPPVLDSDGSFFLYSKLTVDKSRWQQGNVFSCSVMHEALHNHYTQKSLSLSPGK

SEQ ID NO: 64 - protein, 485 aa, synthetic construct
EVQLLESGGGLVQPGGSLKLSCAASGFTFNTYAMNWVRQAPGKGLEWVARIRSKYNNYATYYADSVKDRFTISRDDSKNTAYLQMNNLKTEDTAVYYCVRHGNFGNSYVSWFAYWGQGTLVTVSSGGGGSGGGGSGGGGSELVVTQEPSLTVSPGGTVTLTCRSSTGAVTTSNYANWVQQKPGQAPRGLIGGTNKRAPGTPARFSGSLLGGKAALTLSGVQPEDEAEYYCALWYSNPWVFGGGTKLTVLGGGGSPKSSDKTHTCPPCPAPEAAGGPSVFLFPPKPKDTLMISRTPEVTCVVVDVSHEDPEVKFNWYVDGVEVHNAKTKPREEQYNSTYRVVSVLTVLHQDWLNGKEYKCKVSNKALPAPIEKTISKAKGQPREPQVYTLPPCREEMTKNQVSLWCLVKGFYPSDIAVEWESNGQPENNYKTTPPVLDSDGSFFLYSKLTVDKSRWQQGNVFSCSVMHEALHNHYTQKSLSLSPGK

SEQ ID NO: 65 - protein, 485 aa, synthetic construct
EVQLLESGGGLVQPGGSLKLSCAASGFTFNTYAMNWVRQAPGKGLEWVARIRSKYNNYATYYADSVKDRFTISRDDSKNTAYLQMNNLKTEDTAVYYCVRHGMFGNSYVSWFAYWGQGTLVTVSSGGGGSGGGGSGGGGSELVVTQEPSLTVSPGGTVTLTCRSSTGAVTTSNYANWVQQKPGQAPRGLIGGTNKRAPGTPARFSGSLLGGKAALTLSGVQPEDEAEYYCALWYPNPWVFGGGTKLTVLGGGGSPKSSDKTHTCPPCPAPEAAGGPSVFLFPPKPKDTLMISRTPEVTCVVVDVSHEDPEVKFNWYVDGVEVHNAKTKPREEQYNSTYRVVSVLTVLHQDWLNGKEYKCKVSNKALPAPIEKTISKAKGQPREPQVYTLPPCREEMTKNQVSLWCLVKGFYPSDIAVEWESNGQPENNYKTTPPVLDSDGSFFLYSKLTVDKSRWQQGNVFSCSVMHEALHNHYTQKSLSLSPGK

SEQ ID NO: 66 - protein, 485 aa, synthetic construct
EVQLLESGGGLVQPGGSLKLSCAASGFTFNTYAMNWVRQAPGKGLEWVARIRSKYNNYATYYADSVKDRFTISRDDSKNTAYLQMNNLKTEDTAVYYCVRHGNFGNSYVSWFLYWGQGTLVTVSSGGGGSGGGGSGGGGSELVVTQEPSLTVSPGGTVTLTCRSSTGAVTTSNYANWVQQKPGQAPRGLIGGTNKRAPGTPARFSGSLLGGKAALTLSGVQPEDEAEYYCALWYPNPWVFGGGTKLTVLGGGGSPKSSDKTHTCPPCPAPEAAGGPSVFLFPPKPKDTLMISRTPEVTCVVVDVSHEDPEVKFNWYVDGVEVHNAKTKPREEQYNSTYRVVSVLTVLHQDWLNGKEYKCKVSNKALPAPIEKTISKAKGQPREPQVYTLPPCREEMTKNQVSLWCLVKGFYPSDIAVEWESNGQPENNYKTTPPVLDSDGSFFLYSKLTVDKSRWQQGNVFSCSVMHEALHNHYTQKSLSLSPGK

SEQ ID NO: 67 - protein, 485 aa, synthetic construct
EVQLLESGGGLVQPGGSLKLSCAASGFTFNTYAMNWVRQAPGKGLEWVARIRSKYNNYATYYADSVKDRFTISRDDSKNTAYLQMNNLKTEDTAVYYCVRHGNFGNSYVSWFAYWGQGTLVTVSSGGGGSGGGGSGGGGSELVVTQEPSLTVSPGGTVTLTCRSSTGAVTTSNYANWVQQKPGQAPRGLIGGTNKRAPGTPARFSGSLLGGKAALTLSGVQPEDEAEYYCALWYPNDWVFGGGTKLTVLGGGGSPKSSDKTHTCPPCPAPEAAGGPSVFLFPPKPKDTLMISRTPEVTCVVVDVSHEDPEVKFNWYVDGVEVHNAKTKPREEQYNSTYRVVSVLTVLHQDWLNGKEYKCKVSNKALPAPIEKTISKAKGQPREPQVYTLPPCREEMTKNQVSLWCLVKGFYPSDIAVEWESNGQPENNYKTTPPVLDSDGSFFLYSKLTVDKSRWQQGNVFSCSVMHEALHNHYTQKSLSLSPGK

SEQ ID NO: 68 - protein, 485 aa, synthetic construct
EVQLLESGGGLVQPGGSLKLSCAASGFTFNTYAMNWVRQAPGKGLEWVARIRSKYNNYATYYADSVKDRFTISRDDSKNTAYLQMNNLKTEDTAVYYCVRHGNFGNDYVSWFAYWGQGTLVTVSSGGGGSGGGGSGGGGSELVVTQEPSLTVSPGGTVTLTCRSSTGAVTTSNYANWVQQKPGQAPRGLIGGTNKRAPGTPARFSGSLLGGKAALTLSGVQPEDEAEYYCALWYSNPWVFGGGTKLTVLGGGGSPKSSDKTHTCPPCPAPEAAGGPSVFLFPPKPKDTLMISRTPEVTCVVVDVSHEDPEVKFNWYVDGVEVHNAKTKPREEQYNSTYRVVSVLTVLHQDWLNGKEYKCKVSNKALPAPIEKTISKAKGQPREPQVYTLPPCREEMTKNQVSLWCLVKGFYPSDIAVEWESNGQPENNYKTTPPVLDSDGSFFLYSKLTVDKSRWQQGNVFSCSVMHEALHNHYTQKSLSLSPGK

SEQ ID NO: 69 - protein, 451 aa, synthetic construct
QVQLQQSGSELKKPGASVKVSCKASGYTFTNYGMNWVKQAPGQGLKWMGWINTYTGEPTYTDDFKGRFAFSLDTSVSTAYLQISSLKADDTAVYFCARGGFGSSYWYFDVWGQGSLVTVSSASTKGPSVFPLAPSSKSTSGGTAALGCLVKDYFPEPVTVSWNSGALTSGVHTFPAVLQSSGLYSLSSVVTVPSSSLGTQTYICNVNHKPSNTKVDKKVEPKSSDKTHTCPPCPAPEAAGGPSVFLFPPKPKDTLMISRTPEVTCVVVDVSHEDPEVKFNWYVDGVEVHNAKTKPREEQYNSTYRVVSVLTVLHQDWLNGKEYKCKVSNKALPAPIEKTISKAKGQPREPQVCTLPPSREEMTKNQVSLSCAVKGFYPSDIAVEWESNGQPENNYKTTPPVLDSDGSFFLVSKLTVDKSRWQQGNVFSCSVMHEALHNHYTQKSLSLSPGK

SEQ ID NO: 70 - protein, 214 aa, synthetic construct
DIQLTQSPSSLSASVGDRVSITCKASQDVSIAVAWYQQKPGKAPKLLIYSASYRYTGVPDRFSGSGSGTDFTLTISSLQPEDFAVYYCQQHYITPLTFGAGTKVEIKRTVAAPSVFIFPPSDEQLKSGTASVVCLLNNFYPREAKVQWKVDNALQSGNSQESVTEQDSKDSTYSLSSTLTLSKADYEKHKVYACEVTHQGLSSPVTKSFNRGEC

SEQ ID NO: 71 - protein, 449 aa, synthetic construct
QVQLVQSGAEVKKPGASVKVSCKASGYSFTGYYMHWVRQAPGQGLEWIGRINPYNGATTYSQNFKDRATMTVDTSISTAYMELSRLRSDDTAVYYCVPTGMGYFLMDYWGQGTLVTVSSASTKGPSVFPLAPSSKSTSGGTAALGCLVKDYFPEPVTVSWNSGALTSGVHTFPAVLQSSGLYSLSSVVTVPSSSLGTQTYICNVNHKPSNTKVDKKVEPKSCDKTHTCPPCPAPEAAGGPSVFLFPPKPKDTLMISRTPEVTCVVVDVSHEDPEVKFNWYVDGVEVHNAKTKPREEQYNSTYRVVSVLTVLHQDWLNGKEYKCKVSNKALPAPIEKTISKAKGQPREPQVCTLPPSREEMTKNQVSLSCAVKGFYPSDIAVEWESNGQPENNYKTTPPVLDSDGSFFLVSKLTVDKSRWQQGNVFSCSVMHEALHNHYTQKSLSLSPGK

SEQ ID NO: 72 - protein, 213 aa, synthetic construct
DIQLTQSPSFLSASVGDRVTITCKASQDVGSAVVWYQQKPGKAPKLLIYWASTRHTGVPSRFSGSGSGTEFTLTISSLQPEDFATYFCQQFTSYPTFGQGTKLEIKRTVAAPSVFIFPPSDEQLKSGTASVVCLLNNFYPREAKVQWKVDNALQSGNSQESVTEQDSKDSTYSLSSTLTLSKADYEKHKVYACEVTHQGLSSPVTKSFNRGEC

SEQ ID NO: 73 - protein, 207 aa, synthetic construct
MQSGTHWRVLGLCLLSVGVWGQDGNEEMGGITQTPYKVSISGTTVILTCPQYPGSEILWQHNDKNIGGDEDDKNIGSDEDHLSLKEFSELEQSGYYVCYPRGSKPEDANFYLYLRARVCENCMEMDVMSVATIVIVDICITGGLLLLVYYWSKNRKAKAKPVTRGAGAGGRQRGQNKERPPPVPNPDYEPIRKGQRDLYSGLNQRRI

SEQ ID NO: 74 - protein, 16 aa, synthetic construct
VRHGMFGNSYVSWFAY

SEQ ID NO: 75 - protein, 16 aa, synthetic construct
VRHGNFGNEYVSWFAY

SEQ ID NO: 76 - protein, 16 aa, synthetic construct
VRHGNFGNPYVSWFAY

SEQ ID NO: 77 - protein, 16 aa, synthetic construct
VRHGNFGNVYVSWFAY

SEQ ID NO: 78 - protein, 16 aa, synthetic construct
VRHGNFGNYYVSWFAY

SEQ ID NO: 79 - protein, 16 aa, synthetic construct
VRHGNFGNSEVSWFAY

SEQ ID NO: 80 - protein, 16 aa, synthetic construct
VRHGNFGNSYHSWFAY

SEQ ID NO: 81 - protein, 16 aa, synthetic construct
VRHGNFGNSYSSWFAY

SEQ ID NO: 82 - protein, 16 aa, synthetic construct
VRHGNFGNSYVSWFAG

SEQ ID NO: 83 - protein, 16 aa, synthetic construct
VRHGNFGNSYVSWFAM

SEQ ID NO: 84 - protein, 16 aa, synthetic construct
VRHGMFGNSYVSWFAY

SEQ ID NO: 85 - protein, 16 aa, synthetic construct
VRHGNFGNSYVSWFLY

SEQ ID NO: 86 - protein, 16 aa, synthetic construct
VRHGNFGNDYVSWFAY

SEQ ID NO: 87 - protein, 9 aa, synthetic construct
ALWYPNLWV

SEQ ID NO: 88 - protein, 9 aa, synthetic construct
ALWYSNPWV

SEQ ID NO: 89 - protein, 9 aa, synthetic construct
ALWYPNPWV

SEQ ID NO: 90 - protein, 9 aa, synthetic construct
ALWYPNPWV

SEQ ID NO: 91 - protein, 9 aa, synthetic construct
ALWYPNDWV

SEQ ID NO: 92 - protein, 9 aa, synthetic construct
ALWYSNPWV

SEQ ID NO: 93 - protein, 330 aa, synthetic construct
ASTKGPSVFPLAPSSKSTSGGTAALGCLVKDYFPEPVTVSWNSGALTSGVHTFPAVLQSSGLYSLSSVVTVPSSSLGTQTYICNVNHKPSNTKVDKKVEPKSCDKTHTCPPCPAPELLGGPSVFLFPPKPKDTLMISRTPEVTCVVVDVSHEDPEVKFNWYVDGVEVHNAKTKPREEQYNSTYRVVSVLTVLHQDWLNGKEYKCKVSNKALPAPIEKTISKAKGQPREPQVYTLPPSREEMTKNQVSLTCLVKGFYPSDIAVEWESNGQPENNYKTTPPVLDSDGSFFLYSKLTVDKSRWQQGNVFSCSVMHEALHNHYTQKSLSLSPGK

SEQ ID NO: 94 - protein, 107 aa, synthetic construct [sequence omitted]

SEQ ID NO: 95 - protein, 455 aa, synthetic construct; identical to SEQ ID NO: 37

SEQ ID NO: 96 - protein, 455 aa, synthetic construct; identical to SEQ ID NO: 34

SEQ ID NO: 97 - protein, 455 aa, synthetic construct; identical to SEQ ID NO: 35

SEQ ID NO: 98 - protein, 455 aa, synthetic construct
EVQLLESGGGLVQPGGSLKLSCAASGFTFNTYAMNWVRQAPGKGLEWVARIRSKYNNYATYYADSVKDRFTISRDDSKNTAYLQMNNLKTEDTAVYYCVRHGNFGNDYVSWFAYWGQGTLVTVSSASTKGPSVFPLAPSSKSTSGGTAALGCLVKDYFPEPVTVSWNSGALTSGVHTFPAVLQSSGLYSLSSVVTVPSSSLGTQTYICNVNHKPSNTKVDKKVEPKSCDKTHTCPPCPAPELLGGPSVFLFPPKPKDTLMISRTPEVTCVVVDVSHEDPEVKFNWYVDGVEVHNAKTKPREEQYNSTYRVVSVLTVLHQDWLNGKEYKCKVSNKALPAPIEKTISKAKGQPREPQVYTLPPSREEMTKNQVSLTCLVKGFYPSDIAVEWESNGQPENNYKTTPPVLDSDGSFFLYSKLTVDKSRWQQGNVFSCSVMHEALHNHYTQKSLSLSPGK

SEQ ID NO: 99 - protein, 249 aa, synthetic construct
EVQLLESGGGLVQPGGSLKLSCAASGFTFNTYAMNWVRQAPGKGLEWVARIRSKYNNYATYYADSVKDRFTISRDDSKNTAYLQMNNLKTEDTAVYYCVRHGMFGNSYVSWFAYWGQGTLVTVSSGGGGSGGGGSGGGGSELVVTQEPSLTVSPGGTVTLTCRSSTGAVTTSNYANWVQQKPGQAPRGLIGGTNKRAPGTPARFSGSLLGGKAALTLSGVQPEDEAEYYCALWYSNLWVFGGGTKLTVL

SEQ ID NO: 100 - protein, 249 aa, synthetic construct
EVQLLESGGGLVQPGGSLKLSCAASGFTFNTYAMNWVRQAPGKGLEWVARIRSKYNNYATYYADSVKDRFTISRDDSKNTAYLQMNNLKTEDTAVYYCVRHGNFGNEYVSWFAYWGQGTLVTVSSGGGGSGGGGSGGGGSELVVTQEPSLTVSPGGTVTLTCRSSTGAVTTSNYANWVQQKPGQAPRGLIGGTNKRAPGTPARFSGSLLGGKAALTLSGVQPEDEAEYYCALWYSNLWVFGGGTKLTVL

SEQ ID NO: 101 - protein, 249 aa, synthetic construct
EVQLLESGGGLVQPGGSLKLSCAASGFTFNTYAMNWVRQAPGKGLEWVARIRSKYNNYATYYADSVKDRFTISRDDSKNTAYLQMNNLKTEDTAVYYCVRHGNFGNPYVSWFAYWGQGTLVTVSSGGGGSGGGGSGGGGSELVVTQEPSLTVSPGGTVTLTCRSSTGAVTTSNYANWVQQKPGQAPRGLIGGTNKRAPGTPARFSGSLLGGKAALTLSGVQPEDEAEYYCALWYSNLWVFGGGTKLTVL

SEQ ID NO: 102 - protein, 249 aa, synthetic construct
EVQLLESGGGLVQPGGSLKLSCAASGFTFNTYAMNWVRQAPGKGLEWVARIRSKYNNYATYYADSVKDRFTISRDDSKNTAYLQMNNLKTEDTAVYYCVRHGNFGNVYVSWFAYWGQGTLVTVSSGGGGSGGGGSGGGGSELVVTQEPSLTVSPGGTVTLTCRSSTGAVTTSNYANWVQQKPGQAPRGLIGGTNKRAPGTPARFSGSLLGGKAALTLSGVQPEDEAEYYCALWYSNLWVFGGGTKLTVL

SEQ ID NO: 103 - protein, 249 aa, synthetic construct
EVQLLESGGGLVQPGGSLKLSCAASGFTFNTYAMNWVRQAPGKGLEWVARIRSKYNNYATYYADSVKDRFTISRDDSKNTAYLQMNNLKTEDTAVYYCVRHGNFGNYYVSWFAYWGQGTLVTVSSGGGGSGGGGSGGGGSELVVTQEPSLTVSPGGTVTLTCRSSTGAVTTSNYANWVQQKPGQAPRGLIGGTNKRAPGTPARFSGSLLGGKAALTLSGVQPEDEAEYYCALWYSNLWVFGGGTKLTVL

SEQ ID NO: 104 - protein, 249 aa, synthetic construct
EVQLLESGGGLVQPGGSLKLSCAASGFTFNTYAMNWVRQAPGKGLEWVARIRSKYNNYATYYADSVKDRFTISRDDSKNTAYLQMNNLKTEDTAVYYCVRHGNFGNSEVSWFAYWGQGTLVTVSSGGGGSGGGGSGGGGSELVVTQEPSLTVSPGGTVTLTCRSSTGAVTTSNYANWVQQKPGQAPRGLIGGTNKRAPGTPARFSGSLLGGKAALTLSGVQPEDEAEYYCALWYSNLWVFGGGTKLTVL

SEQ ID NO: 105 - protein, 249 aa, synthetic construct
EVQLLESGGGLVQPGGSLKLSCAASGFTFNTYAMNWVRQAPGKGLEWVARIRSKYNNYATYYADSVKDRFTISRDDSKNTAYLQMNNLKTEDTAVYYCVRHGNFGNSYHSWFAYWGQGTLVTVSSGGGGSGGGGSGGGGSELVVTQEPSLTVSPGGTVTLTCRSSTGAVTTSNYANWVQQKPGQAPRGLIGGTNKRAPGTPARFSGSLLGGKAALTLSGVQPEDEAEYYCALWYSNLWVFGGGTKLTVL

SEQ ID NO: 106 - protein, 249 aa, synthetic construct
EVQLLESGGGLVQPGGSLKLSCAASGFTFNTYAMNWVRQAPGKGLEWVARIRSKYNNYATYYADSVKDRFTISRDDSKNTAYLQMNNLKTEDTAVYYCVRHGNFGNSYQSWFAYWGQGTLVTVSSGGGGSGGGGSGGGGSELVVTQEPSLTVSPGGTVTLTCRSSTGAVTTSNYANWVQQKPGQAPRGLIGGTNKRAPGTPARFSGSLLGGKAALTLSGVQPEDEAEYYCALWYSNLWVFGGGTKLTVL

SEQ ID NO: 107 - protein, 249 aa, synthetic construct
EVQLLESGGGLVQPGGSLKLSCAASGFTFNTYAMNWVRQAPGKGLEWVARIRSKYNNYATYYADSVKDRFTISRDDSKNTAYLQMNNLKTEDTAVYYCVRHGNFGNSYSSWFAYWGQGTLVTVSSGGGGSGGGGSGGGGSELVVTQEPSLTVSPGGTVTLTCRSSTGAVTTSNYANWVQQKPGQAPRGLIGGTNKRAPGTPARFSGSLLGGKAALTLSGVQPEDEAEYYCALWYSNLWVFGGGTKLTVL

SEQ ID NO: 108 - protein, 249 aa, synthetic construct
EVQLLESGGGLVQPGGSLKLSCAASGFTFNTYAMNWVRQAPGKGLEWVARIRSKYNNYATYYADSVKDRFTISRDDSKNTAYLQMNNLKTEDTAVYYCVRHGNFGNSYVSWFLYWGQGTLVTVSSGGGGSGGGGSGGGGSELVVTQEPSLTVSPGGTVTLTCRSSTGAVTTSNYANWVQQKPGQAPRGLIGGTNKRAPGTPARFSGSLLGGKAALTLSGVQPEDEAEYYCALWYSNLWVFGGGTKLTVL

SEQ ID NO: 109 - protein, 249 aa, synthetic construct
EVQLLESGGGLVQPGGSLKLSCAASGFTFNTYAMNWVRQAPGKGLEWVARIRSKYNNYATYYADSVKDRFTISRDDSKNTAYLQMNNLKTEDTAVYYCVRHGNFGNSYVSWFAGWGQGTLVTVSSGGGGSGGGGSGGGGSELVVTQEPSLTVSPGGTVTLTCRSSTGAVTTSNYANWVQQKPGQAPRGLIGGTNKRAPGTPARFSGSLLGGKAALTLSGVQPEDEAEYYCALWYSNLWVFGGGTKLTVL

SEQ ID NO: 110 - protein, 249 aa, synthetic construct
EVQLLESGGGLVQPGGSLKLSCAASGFTFNTYAMNWVRQAPGKGLEWVARIRSKYNNYATYYADSVKDRFTISRDDSKNTAYLQMNNLKTEDTAVYYCVRHGNFGNSYVSWFAMWGQGTLVTVSSGGGGSGGGGSGGGGSELVVTQEPSLTVSPGGTVTLTCRSSTGAVTTSNYANWVQQKPGQAPRGLIGGTNKRAPGTPARFSGSLLGGKAALTLSGVQPEDEAEYYCALWYSNLWVFGGGTKLTVL

SEQ ID NO: 111 - protein, 249 aa, synthetic construct
EVQLLESGGGLVQPGGSLKLSCAASGFTFNTYAMNWVRQAPGKGLEWVARIRSKYNNYATYYADSVKDRFTISRDDSKNTAYLQMNNLKTEDTAVYYCVRHGNFGNSYVSWFAYWGQGTLVTVSSGGGGSGGGGSGGGGSELVVTQEPSLTVSPGGTVTLTCRSSTGAVTTSNYANWVQQKPGQAPRGLIGGTNKRAPGTPARFSGSLLGGKAALTLSGVQPEDEAEYYCALWYPNLWVFGGGTKLTVL

SEQ ID NO: 112 - protein, 249 aa, synthetic construct
EVQLLESGGGLVQPGGSLKLSCAASGFTFNTYAMNWVRQAPGKGLEWVARIRSKYNNYATYYADSVKDRFTISRDDSKNTAYLQMNNLKTEDTAVYYCVRHGNFGNSYVSWFAYWGQGTLVTVSSGGGGSGGGGSGGGGSELVVTQEPSLTVSPGGTVTLTCRSSTGAVTTSNYANWVQQKPGQAPRGLIGGTNKRAPGTPARFSGSLLGGKAALTLSGVQPEDEAEYYCALWYSNDWVFGGGTKLTVL

SEQ ID NO: 113 - protein, 249 aa, synthetic construct
EVQLLESGGGLVQPGGSLKLSCAASGFTFNTYAMNWVRQAPGKGLEWVARIRSKYNNYATYYADSVKDRFTISRDDSKNTAYLQMNNLKTEDTAVYYCVRHGNFGNSYVSWFAYWGQGTLVTVSSGGGGSGGGGSGGGGSELVVTQEPSLTVSPGGTVTLTCRSSTGAVTTSNYANWVQQKPGQAPRGLIGGTNKRAPGTPARFSGSLLGGKAALTLSGVQPEDEAEYYCALWYSNPWVFGGGTKLTVL

SEQ ID NO: 114 - protein, 249 aa, synthetic construct
EVQLLESGGGLVQPGGSLKLSCAASGFTFNTYAMNWVRQAPGKGLEWVARIRSKYNNYATYYADSVKDRFTISRDDSKNTAYLQMNNLKTEDTAVYYCVRHGMFGNSYVSWFAYWGQGTLVTVSSGGGGSGGGGSGGGGSELVVTQEPSLTVSPGGTVTLTCRSSTGAVTTSNYANWVQQKPGQAPRGLIGGTNKRAPGTPARFSGSLLGGKAALTLSGVQPEDEAEYYCALWYPNPWVFGGGTKLTVL

SEQ ID NO: 115 - protein, 249 aa, synthetic construct
EVQLLESGGGLVQPGGSLKLSCAASGFTFNTYAMNWVRQAPGKGLEWVARIRSKYNNYATYYADSVKDRFTISRDDSKNTAYLQMNNLKTEDTAVYYCVRHGNFGNSYVSWFLYWGQGTLVTVSSGGGGSGGGGSGGGGSELVVTQEPSLTVSPGGTVTLTCRSSTGAVTTSNYANWVQQKPGQAPRGLIGGTNKRAPGTPARFSGSLLGGKAALTLSGVQPEDEAEYYCALWYPNPWVFGGGTKLTVL

SEQ ID NO: 116 - protein, 249 aa, synthetic construct
EVQLLESGGGLVQPGGSLKLSCAASGFTFNTYAMNWVRQAPGKGLEWVARIRSKYNNYATYYADSVKDRFTISRDDSKNTAYLQMNNLKTEDTAVYYCVRHGNFGNSYVSWFAYWGQGTLVTVSSGGGGSGGGGSGGGGSELVVTQEPSLTVSPGGTVTLTCRSSTGAVTTSNYANWVQQKPGQAPRGLIGGTNKRAPGTPARFSGSLLGGKAALTLSGVQPEDEAEYYCALWYPNDWVFGGGTKLTVL

SEQ ID NO: 117 - protein, 249 aa, synthetic construct
EVQLLESGGGLVQPGGSLKLSCAASGFTFNTYAMNWVRQAPGKGLEWVARIRSKYNNYATYYADSVKDRFTISRDDSKNTAYLQMNNLKTEDTAVYYCVRHGNFGNDYVSWFAYWGQGTLVTVSSGGGGSGGGGSGGGGSELVVTQEPSLTVSPGGTVTLTCRSSTGAVTTSNYANWVQQKPGQAPRGLIGGTNKRAPGTPARFSGSLLGGKAALTLSGVQPEDEAEYYCALWYSNPWVFGGGTKLTVL

SEQ ID NO: 118 - protein, 231 aa, synthetic construct
PKSSDKTHTCPPCPAPEAAGGPSVFLFPPKPKDTLMISRTPEVTCVVVDVSHEDPEVKFNWYVDGVEVHNAKTKPREEQYNSTYRVVSVLTVLHQDWLNGKEYKCKVSNKALPAPIEKTISKAKGQPREPQVYTLPPCREEMTKNQVSLWCLVKGFYPSDIAVEWESNGQPENNYKTTPPVLDSDGSFFLYSKLTVDKSRWQQGNVFSCSVMHEALHNHYTQKSLSLSPGK

SEQ ID NO: 119 - protein, 216 aa, synthetic construct
ELVVTQEPSLTVSPGGTVTLTCRSSTGAVTTSNYANWVQQKPGQAPRGLIGGTNKRAPGTPARFSGSLLGGKAALTLSGVQPEDEAEYYCALWYPNPWVFGGGTKLTVLRTVAAPSVFIFPPSDEQLKSGTASVVCLLNNFYPREAKVQWKVDNALQSGNSQESVTEQDSKDSTYSLSSTLTLSKADYEKHKVYACEVTHQGLSSPVTKSFNRGEC

SEQ ID NO: 120 - protein, 216 aa, synthetic construct; identical to SEQ ID NO: 119

SEQ ID NO: 121 - protein, 216 aa, synthetic construct
ELVVTQEPSLTVSPGGTVTLTCRSSTGAVTTSNYANWVQQKPGQAPRGLIGGTNKRAPGTPARFSGSLLGGKAALTLSGVQPEDEAEYYCALWYPNDWVFGGGTKLTVLRTVAAPSVFIFPPSDEQLKSGTASVVCLLNNFYPREAKVQWKVDNALQSGNSQESVTEQDSKDSTYSLSSTLTLSKADYEKHKVYACEVTHQGLSSPVTKSFNRGEC

SEQ ID NO: 122 - protein, 216 aa, synthetic construct; identical to SEQ ID NO: 48

SEQ ID NO: 123 - protein, 224 aa, synthetic construct
EVQLLESGGGLVQPGGSLKLSCAASGFTFNTYAMNWVRQAPGKGLEWVARIRSKYNNYATYYADSVKDRFTISRDDSKNTAYLQMNNLKTEDTAVYYCVRHGMFGNSYVSWFAYWGQGTLVTVSSASTKGPSVFPLAPSSKSTSGGTAALGCLVKDYFPEPVTVSWNSGALTSGVHTFPAVLQSSGLYSLSSVVTVPSSSLGTQTYICNVNHKPSNTKVDKKVE

SEQ ID NO: 124 - protein, 224 aa, synthetic construct
EVQLLESGGGLVQPGGSLKLSCAASGFTFNTYAMNWVRQAPGKGLEWVARIRSKYNNYATYYADSVKDRFTISRDDSKNTAYLQMNNLKTEDTAVYYCVRHGNFGNEYVSWFAYWGQGTLVTVSSASTKGPSVFPLAPSSKSTSGGTAALGCLVKDYFPEPVTVSWNSGALTSGVHTFPAVLQSSGLYSLSSVVTVPSSSLGTQTYICNVNHKPSNTKVDKKVE

SEQ ID NO: 125 - protein, 224 aa, synthetic construct
EVQLLESGGGLVQPGGSLKLSCAASGFTFNTYAMNWVRQAPGKGLEWVARIRSKYNNYATYYADSVKDRFTISRDDSKNTAYLQMNNLKTEDTAVYYCVRHGNFGNPYVSWFAYWGQGTLVTVSSASTKGPSVFPLAPSSKSTSGGTAALGCLVKDYFPEPVTVSWNSGALTSGVHTFPAVLQSSGLYSLSSVVTVPSSSLGTQTYICNVNHKPSNTKVDKKVE

SEQ ID NO: 126 - protein, 224 aa, synthetic construct
EVQLLESGGGLVQPGGSLKLSCAASGFTFNTYAMNWVRQAPGKGLEWVARIRSKYNNYATYYADSVKDRFTISRDDSKNTAYLQMNNLKTEDTAVYYCVRHGNFGNVYVSWFAYWGQGTLVTVSSASTKGPSVFPLAPSSKSTSGGTAALGCLVKDYFPEPVTVSWNSGALTSGVHTFPAVLQSSGLYSLSSVVTVPSSSLGTQTYICNVNHKPSNTKVDKKVE

SEQ ID NO: 127 - protein, 224 aa, synthetic construct
EVQLLESGGGLVQPGGSLKLSCAASGFTFNTYAMNWVRQAPGKGLEWVARIRSKYNNYATYYADSVKDRFTISRDDSKNTAYLQMNNLKTEDTAVYYCVRHGNFGNYYVSWFAYWGQGTLVTVSSASTKGPSVFPLAPSSKSTSGGTAALGCLVKDYFPEPVTVSWNSGALTSGVHTFPAVLQSSGLYSLSSVVTVPSSSLGTQTYICNVNHKPSNTKVDKKVE

SEQ ID NO: 128 - protein, 224 aa, synthetic construct
EVQLLESGGGLVQPGGSLKLSCAASGFTFNTYAMNWVRQAPGKGLEWVARIRSKYNNYATYYADSVKDRFTISRDDSKNTAYLQMNNLKTEDTAVYYCVRHGNFGNSEVSWFAYWGQGTLVTVSSASTKGPSVFPLAPSSKSTSGGTAALGCLVKDYFPEPVTVSWNSGALTSGVHTFPAVLQSSGLYSLSSVVTVPSSSLGTQTYICNVNHKPSNTKVDKKVE

SEQ ID NO: 129 - protein, 224 aa, synthetic construct
EVQLLESGGGLVQPGGSLKLSCAASGFTFNTYAMNWVRQAPGKGLEWVARIRSKYNNYATYYADSVKDRFTISRDDSKNTAYLQMNNLKTEDTAVYYCVRHGNFGNSYHSWFAYWGQGTLVTVSSASTKGPSVFPLAPSSKSTSGGTAALGCLVKDYFPEPVTVSWNSGALTSGVHTFPAVLQSSGLYSLSSVVTVPSSSLGTQTYICNVNHKPSNTKVDKKVE

SEQ ID NO: 130 - protein, 224 aa, synthetic construct
EVQLLESGGGLVQPGGSLKLSCAASGFTFNTYAMNWVRQAPGKGLEWVARIRSKYNNYATYYADSVKDRFTISRDDSKNTAYLQMNNLKTEDTAVYYCVRHGNFGNSYQSWFAYWGQGTLVTVSSASTKGPSVFPLAPSSKSTSGGTAALGCLVKDYFPEPVTVSWNSGALTSGVHTFPAVLQSSGLYSLSSVVTVPSSSLGTQTYICNVNHKPSNTKVDKKVE

SEQ ID NO: 131 - protein, 224 aa, synthetic construct
EVQLLESGGGLVQPGGSLKLSCAASGFTFNTYAMNWVRQAPGKGLEWVARIRSKYNNYATYYADSVKDRFTISRDDSKNTAYLQMNNLKTEDTAVYYCVRHGNFGNSYSSWFAYWGQGTLVTVSSASTKGPSVFPLAPSSKSTSGGTAALGCLVKDYFPEPVTVSWNSGALTSGVHTFPAVLQSSGLYSLSSVVTVPSSSLGTQTYICNVNHKPSNTKVDKKVE

SEQ ID NO: 132 - protein, 224 aa, synthetic construct
EVQLLESGGGLVQPGGSLKLSCAASGFTFNTYAMNWVRQAPGKGLEWVARIRSKYNNYATYYADSVKDRFTISRDDSKNTAYLQMNNLKTEDTAVYYCVRHGNFGNSYVSWFLYWGQGTLVTVSSASTKGPSVFPLAPSSKSTSGGTAALGCLVKDYFPEPVTVSWNSGALTSGVHTFPAVLQSSGLYSLSSVVTVPSSSLGTQTYICNVNHKPSNTKVDKKVE

SEQ ID NO: 133 - protein, 224 aa, synthetic construct
EVQLLESGGGLVQPGGSLKLSCAASGFTFNTYAMNWVRQAPGKGLEWVARIRSKYNNYATYYADSVKDRFTISRDDSKNTAYLQMNNLKTEDTAVYYCVRHGNFGNSYVSWFAGWGQGTLVTVSSASTKGPSVFPLAPSSKSTSGGTAALGCLVKDYFPEPVTVSWNSGALTSGVHTFPAVLQSSGLYSLSSVVTVPSSSLGTQTYICNVNHKPSNTKVDKKVE

SEQ ID NO: 134 - protein, 224 aa, synthetic construct
EVQLLESGGGLVQPGGSLKLSCAASGFTFNTYAMNWVRQAPGKGLEWVARIRSKYNNYATYYADSVKDRFTISRDDSKNTAYLQMNNLKTEDTAVYYCVRHGNFGNSYVSWFAMWGQGTLVTVSSASTKGPSVFPLAPSSKSTSGGTAALGCLVKDYFPEPVTVSWNSGALTSGVHTFPAVLQSSGLYSLSSVVTVPSSSLGTQTYICNVNHKPSNTKVDKKVE

SEQ ID NO: 135 - protein, 224 aa, synthetic construct
EVQLLESGGGLVQPGGSLKLSCAASGFTFNTYAMNWVRQAPGKGLEWVARIRSKYNNYATYYADSVKDRFTISRDDSKNTAYLQMNNLKTEDTAVYYCVRHGNFGNSYVSWFAYWGQGTLVTVSSASTKGPSVFPLAPSSKSTSGGTAALGCLVKDYFPEPVTVSWNSGALTSGVHTFPAVLQSSGLYSLSSVVTVPSSSLGTQTYICNVNHKPSNTKVDKKVE

SEQ ID NO: 136 - protein, 224 aa, synthetic construct; identical to SEQ ID NO: 135

SEQ ID NO: 137 - protein, 224 aa, synthetic construct; identical to SEQ ID NO: 135

SEQ ID NO: 138 - protein, 224 aa, synthetic construct; identical to SEQ ID NO: 123

SEQ ID NO: 139 - protein, 224 aa, synthetic construct; identical to SEQ ID NO: 132

SEQ ID NO: 140 - protein, 224 aa, synthetic construct; identical to SEQ ID NO: 135

SEQ ID NO: 141 - protein, 224 aa, synthetic construct
EVQLLESGGGLVQPGGSLKLSCAASGFTFNTYAMNWVRQAPGKGLEWVARIRSKYNNYATYYADSVKDRFTISRDDSKNTAYLQMNNLKTEDTAVYYCVRHGNFGNDYVSWFAYWGQGTLVTVSSASTKGPSVFPLAPSSKSTSGGTAALGCLVKDYFPEPVTVSWNSGALTSGVHTFPAVLQSSGLYSLSSVVTVPSSSLGTQTYICNVNHKPSNTKVDKKVE

SEQ ID NO: 142 - protein, 478 aa, synthetic construct
ELVVTQEPSLTVSPGGTVTLTCRSSTGAVTTSNYANWVQQKPGQAPRGLIGGTNKRAPGTPARFSGSLLGGKAALTLSGVQPEDEAEYYCALWYSNLWVFGGGTKLTVLRTVAAPSVFIFPPSDEQLKSGTASVVCLLNNFYPREAKVQWKVDNALQSGNSQESVTEQDSKDSTYSLSSTLTLSKADYEKHKVYACEVTHQGLSSPVTKSFNRGECGGGGSEGKSSGSGSESKSTEGKSSGSGSESKSTGGGGSEVQLLESGGGLVQPGGSLKLSCAASGFTFNTYAMNWVRQAPGKGLEWVARIRSKYNNYATYYADSVKDRFTISRDDSKNTAYLQMNNLKTEDTAVYYCVRHGMFGNSYVSWFAYWGQGTLVTVSSASTKGPSVFPLAPSSKSTSGGTAALGCLVKDYFPEPVTVSWNSGALTSGVHTFPAVLQSSGLYSLSSVVTVPSSSLGTQTYICNVNHKPSNTKVDKKVE

SEQ ID NO: 143 - protein, 478 aa, synthetic construct
ELVVTQEPSLTVSPGGTVTLTCRSSTGAVTTSNYANWVQQKPGQAPRGLIGGTNKRAPGTPARFSGSLLGGKAALTLSGVQPEDEAEYYCALWYSNLWVFGGGTKLTVLRTVAAPSVFIFPPSDEQLKSGTASVVCLLNNFYPREAKVQWKVDNALQSGNSQESVTEQDSKDSTYSLSSTLTLSKADYEKHKVYACEVTHQGLSSPVTKSFNRGECGGGGSEGKSSGSGSESKSTEGKSSGSGSESKSTGGGGSEVQLLESGGGLVQPGGSLKLSCAASGFTFNTYAMNWVRQAPGKGLEWVARIRSKYNNYATYYADSVKDRFTISRDDSKNTAYLQMNNLKTEDTAVYYCVRHGNFGNEYVSWFAYWGQGTLVTVSSASTKGPSVFPLAPSSKSTSGGTAALGCLVKDYFPEPVTVSWNSGALTSGVHTFPAVLQSSGLYSLSSVVTVPSSSLGTQTYICNVNHKPSNTKVDKKVE

SEQ ID NO: 144 - protein, 478 aa, synthetic construct
ELVVTQEPSLTVSPGGTVTLTCRSSTGAVTTSNYANWVQQKPGQAPRGLIGGTNKRAPGTPARFSGSLLGGKAALTLSGVQPEDEAEYYCALWYSNLWVFGGGTKLTVLRTVAAPSVFIFPPSDEQLKSGTASVVCLLNNFYPREAKVQWKVDNALQSGNSQESVTEQDSKDSTYSLSSTLTLSKADYEKHKVYACEVTHQGLSSPVTKSFNRGECGGGGSEGKSSGSGSESKSTEGKSSGSGSESKSTGGGGSEVQLLESGGGLVQPGGSLKLSCAASGFTFNTYAMNWVRQAPGKGLEWVARIRSKYNNYATYYADSVKDRFTISRDDSKNTAYLQMNNLKTEDTAVYYCVRHGNFGNPYVSWFAYWGQGTLVTVSSASTKGPSVFPLAPSSKSTSGGTAALGCLVKDYFPEPVTVSWNSGALTSGVHTFPAVLQSSGLYSLSSVVTVPSSSLGTQTYICNVNHKPSNTKVDKKVE

SEQ ID NO: 145 - protein, 478 aa, synthetic construct
ELVVTQEPSLTVSPGGTVTLTCRSSTGAVTTSNYANWVQQKPGQAPRGLIGGTNKRAPGTPARFSGSLLGGKAALTLSGVQPEDEAEYYCALWYSNLWVFGGGTKLTVLRTVAAPSVFIFPPSDEQLKSGTASVVCLLNNFYPREAKVQWKVDNALQSGNSQESVTEQDSKDSTYSLSSTLTLSKADYEKHKVYACEVTHQGLSSPVTKSFNRGECGGGGSEGKSSGSGSESKSTEGKSSGSGSESKSTGGGGSEVQLLESGGGLVQPGGSLKLSCAASGFTFNTYAMNWVRQAPGKGLEWVARIRSKYNNYATYYADSVKDRFTISRDDSKNTAYLQMNNLKTEDTAVYYCVRHGNFGNVYVSWFAYWGQGTLVTVSSASTKGPSVFPLAPSSKSTSGGTAALGCLVKDYFPEPVTVSWNSGALTSGVHTFPAVLQSSGLYSLSSVVTVPSSSLGTQTYICNVNHKPSNTKVDKKVE

SEQ ID NO: 146 - protein, 478 aa, synthetic construct
ELVVTQEPSLTVSPGGTVTLTCRSSTGAVTTSNYANWVQQKPGQAPRGLIGGTNKRAPGTPARFSGSLLGGKAALTLSGVQPEDEAEYYCALWYSNLWVFGGGTKLTVLRTVAAPSVFIFPPSDEQLKSGTASVVCLLNNFYPREAKVQWKVDNALQSGNSQESVTEQDSKDSTYSLSSTLTLSKADYEKHKVYACEVTHQGLSSPVTKSFNRGECGGGGSEGKSSGSGSESKSTEGKSSGSGSESKSTGGGGSEVQLLESGGGLVQPGGSLKLSCAASGFTFNTYAMNWVRQAPGKGLEWVARIRSKYNNYATYYADSVKDRFTISRDDSKNTAYLQMNNLKTEDTAVYYCVRHGNFGNYYVSWFAYWGQGTLVTVSSASTKGPSVFPLAPSSKSTSGGTAALGCLVKDYFPEPVTVSWNSGALTSGVHTFPAVLQSSGLYSLSSVVTVPSSSLGTQTYICNVNHKPSNTKVDKKVE

SEQ ID NO: 147 - protein, 478 aa, synthetic construct
ELVVTQEPSLTVSPGGTVTLTCRSSTGAVTTSNYANWVQQKPGQAPRGLIGGTNKRAPGTPARFSGSLLGGKAALTLSGVQPEDEAEYYCALWYSNLWVFGGGTKLTVLRTVAAPSVFIFPPSDEQLKSGTASVVCLLNNFYPREAKVQWKVDNALQSGNSQESVTEQDSKDSTYSLSSTLTLSKADYEKHKVYACEVTHQGLSSPVTKSFNRGECGGGGSEGKSSGSGSESKSTEGKSSGSGSESKSTGGGGSEVQLLESGGGLVQPGGSLKLSCAASGFTFNTYAMNWVRQAPGKGLEWVARIRSKYNNYATYYADSVKDRFTISRDDSKNTAYLQMNNLKTEDTAVYYCVRHGNFGNSEVSWFAYWGQGTLVTVSSASTKGPSVFPLAPSSKSTSGGTAALGCLVKDYFPEPVTVSWNSGALTSGVHTFPAVLQSSGLYSLSSVVTVPSSSLGTQTYICNVNHKPSNTKVDKKVE

SEQ ID NO: 148 - protein, 478 aa, synthetic construct
ELVVTQEPSLTVSPGGTVTLTCRSSTGAVTTSNYANWVQQKPGQAPRGLIGGTNKRAPGTPARFSGSLLGGKAALTLSGVQPEDEAEYYCALWYSNLWVFGGGTKLTVLRTVAAPSVFIFPPSDEQLKSGTASVVCLLNNFYPREAKVQWKVDNALQSGNSQESVTEQDSKDSTYSLSSTLTLSKADYEKHKVYACEVTHQGLSSPVTKSFNRGECGGGGSEGKSSGSGSESKSTEGKSSGSGSESKSTGGGGSEVQLLESGGGLVQPGGSLKLSCAASGFTFNTYAMNWVRQAPGKGLEWVARIRSKYNNYATYYADSVKDRFTISRDDSKNTAYLQMNNLKTEDTAVYYCVRHGNFGNSYHSWFAYWGQGTLVTVSSASTKGPSVFPLAPSSKSTSGGTAALGCLVKDYFPEPVTVSWNSGALTSGVHTFPAVLQSSGLYSLSSVVTVPSSSLGTQTYICNVNHKPSNTKVDKKVE

SEQ ID NO: 149 - protein, 478 aa, synthetic construct
ELVVTQEPSLTVSPGGTVTLTCRSSTGAVTTSNYANWVQQKPGQAPRGLIGGTNKRAPGTPARFSGSLLGGKAALTLSGVQPEDEAEYYCALWYSNLWVFGGGTKLTVLRTVAAPSVFIFPPSDEQLKSGTASVVCLLNNFYPREAKVQWKVDNALQSGNSQESVTEQDSKDSTYSLSSTLTLSKADYEKHKVYACEVTHQGLSSPVTKSFNRGECGGGGSEGKSSGSGSESKSTEGKSSGSGSESKSTGGGGSEVQLLESGGGLVQPGGSLKLSCAASGFTFNTYAMNWVRQAPGKGLEWVARIRSKYNNYATYYADSVKDRFTISRDDSKNTAYLQMNNLKTEDTAVYYCVRHGNFGNSYQSWFAYWGQGTLVTVSSASTKGPSVFPLAPSSKSTSGGTAALGCLVKDYFPEPVTVSWNSGALTSGVHTFPAVLQSSGLYSLSSVVTVPSSSLGTQTYICNVNHKPSNTKVDKKVE

SEQ ID NO: 150 - protein, 478 aa, synthetic construct
ELVVTQEPSLTVSPGGTVTLTCRSSTGAVTTSNYANWVQQKPGQAPRGLIGGTNKRAPGTPARFSGSLLGGKAALTLSGVQPEDEAEYYCALWYSNLWVFGGGTKLTVLRTVAAPSVFIFPPSDEQLKSGTASVVCLLNNFYPREAKVQWKVDNALQSGNSQESVTEQDSKDSTYSLSSTLTLSKADYEKHKVYACEVTHQGLSSPVTKSFNRGECGGGGSEGKSSGSGSESKSTEGKSSGSGSESKSTGGGGSEVQLLESGGGLVQPGGSLKLSCAASGFTFNTYAMNWVRQAPGKGLEWVARIRSKYNNYATYYADSVKDRFTISRDDSKNTAYLQMNNLKTEDTAVYYCVRHGNFGNSYSSWFAYWGQGTLVTVSSASTKGPSVFPLAPSSKSTSGGTAALGCLVKDYFPEPVTVSWNSGALTSGVHTFPAVLQSSGLYSLSSVVTVPSSSLGTQTYICNVNHKPSNTKVDKKVE

SEQ ID NO: 151 - protein, 478 aa, synthetic construct
ELVVTQEPSLTVSPGGTVTLTCRSSTGAVTTSNYANWVQQKPGQAPRGLIGGTNKRAPGTPARFSGSLLGGKAALTLSGVQPEDEAEYYCALWYSNLWVFGGGTKLTVLRTVAAPSVFIFPPSDEQLKSGTASVVCLLNNFYPREAKVQWKVDNALQSGNSQESVTEQDSKDSTYSLSSTLTLSKADYEKHKVYACEVTHQGLSSPVTKSFNRGECGGGGSEGKSSGSGSESKSTEGKSSGSGSESKSTGGGGSEVQLLESGGGLVQPGGSLKLSCAASGFTFNTYAMNWVRQAPGKGLEWVARIRSKYNNYATYYADSVKDRFTISRDDSKNTAYLQMNNLKTEDTAVYYCVRHGNFGNSYVSWFLYWGQGTLVTVSSASTKGPSVFPLAPSSKSTSGGTAALGCLVKDYFPEPVTVSWNSGALTSGVHTFPAVLQSSGLYSLSSVVTVPSSSLGTQTYICNVNHKPSNTKVDKKVE

SEQ ID NO: 152 - protein, 478 aa, synthetic construct
ELVVTQEPSLTVSPGGTVTLTCRSSTGAVTTSNYANWVQQKPGQAPRGLIGGTNKRAPGTPARFSGSLLGGKAALTLSGVQPEDEAEYYCALWYSNLWVFGGGTKLTVLRTVAAPSVFIFPPSDEQLKSGTASVVCLLNNFYPREAKVQWKVDNALQSGNSQESVTEQDSKDSTYSLSSTLTLSKADYEKHKVYACEVTHQGLSSPVTKSFNRGECGGGGSEGKSSGSGSESKSTEGKSSGSGSESKSTGGGGSEVQLLESGGGLVQPGGSLKLSCAASGFTFNTYAMNWVRQAPGKGLEWVARIRSKYNNYATYYADSVKDRFTISRDDSKNTAYLQMNNLKTEDTAVYYCVRHGNFGNSYVSWFAGWGQGTLVTVSSASTKGPSVFPLAPSSKSTSGGTAALGCLVKDYFPEPVTVSWNSGALTSGVHTFPAVLQSSGLYSLSSVVTVPSSSLGTQTYICNVNHKPSNTKVDKKVE

SEQ ID NO: 153 - protein, 478 aa, synthetic construct
ELVVTQEPSLTVSPGGTVTLTCRSSTGAVTTSNYANWVQQKPGQAPRGLIGGTNKRAPGTPARFSGSLLGGKAALTLSGVQPEDEAEYYCALWYSNLWVFGGGTKLTVLRTVAAPSVFIFPPSDEQLKSGTASVVCLLNNFYPREAKVQWKVDNALQSGNSQESVTEQDSKDSTYSLSSTLTLSKADYEKHKVYACEVTHQGLSSPVTKSFNRGECGGGGSEGKSSGSGSESKSTEGKSSGSGSESKSTGGGGSEVQLLESGGGLVQPGGSLKLSCAASGFTFNTYAMNWVRQAPGKGLEWVARIRSKYNNYATYYADSVKDRFTISRDDSKNTAYLQMNNLKTEDTAVYYCVRHGNFGNSYVSWFAMWGQGTLVTVSSASTKGPSVFPLAPSSKSTSGGTAALGCLVKDYFPEPVTVSWNSGALTSGVHTFPAVLQSSGLYSLSSVVTVPSSSLGTQTYICNVNHKPSNTKVDKKVE

SEQ ID NO: 154 - protein, 478 aa, synthetic construct
ELVVTQEPSLTVSPGGTVTLTCRSSTGAVTTSNYANWVQQKPGQAPRGLIGGTNKRAPGTPARFSGSLLGGKAALTLSGVQPEDEAEYYCALWYPNLWVFGGGTKLTVLRTVAAPSVFIFPPSDEQLKSGTASVVCLLNNFYPREAKVQWKVDNALQSGNSQESVTEQDSKDSTYSLSSTLTLSKADYEKHKVYACEVTHQGLSSPVTKSFNRGECGGGGSEGKSSGSGSESKSTEGKSSGSGSESKSTGGGGSEVQLLESGGGLVQPGGSLKLSCAASGFTFNTYAMNWVRQAPGKGLEWVARIRSKYNNYATYYADSVKDRFTISRDDSKNTAYLQMNNLKTEDTAVYYCVRHGNFGNSYVSWFAYWGQGTLVTVSSASTKGPSVFPLAPSSKSTSGGTAALGCLVKDYFPEPVTVSWNSGALTSGVHTFPAVLQSSGLYSLSSVVTVPSSSLGTQTYICNVNHKPSNTKVDKKVE

SEQ ID NO: 155 - protein, 478 aa, synthetic construct
ELVVTQEPSLTVSPGGTVTLTCRSSTGAVTTSNYANWVQQKPGQAPRGLIGGTNKRAPGTPARFSGSLLGGKAALTLSGVQPEDEAEYYCALWYSNDWVFGGGTKLTVLRTVAAPSVFIFPPSDEQLKSGTASVVCLLNNFYPREAKVQWKVDNALQSGNSQESVTEQDSKDSTYSLSSTLTLSKADYEKHKVYACEVTHQGLSSPVTKSFNRGECGGGGSEGKSSGSGSESKSTEGKSSGSGSESKSTGGGGSEVQLLESGGGLVQPGGSLKLSCAASGFTFNTYAMNWVRQAPGKGLEWVARIRSKYNNYATYYADSVKDRFTISRDDSKNTAYLQMNNLKTEDTAVYYCVRHGNFGNSYVSWFAYWGQGTLVTVSSASTKGPSVFPLAPSSKSTSGGTAALGCLVKDYFPEPVTVSWNSGALTSGVHTFPAVLQSSGLYSLSSVVTVPSSSLGTQTYICNVNHKPSNTKVDKKVE

SEQ ID NO: 156 - protein, 478 aa, synthetic construct
ELVVTQEPSLTVSPGGTVTLTCRSSTGAVTTSNYANWVQQKPGQAPRGLIGGTNKRAPGTPARFSGSLLGGKAALTLSGVQPEDEAEYYCALWYSNPWVFGGGTKLTVLRTVAAPSVFIFPPSDEQLKSGTASVVCLLNNFYPREAKVQWKVDNALQSGNSQESVTEQDSKDSTYSLSSTLTLSKADYEKHKVYACEVTHQGLSSPVTKSFNRGECGGGGSEGKSSGSGSESKSTEGKSSGSGSESKSTGGGGSEVQLLESGGGLVQPGGSLKLSCAASGFTFNTYAMNWVRQAPGKGLEWVARIRSKYNNYATYYADSVKDRFTISRDDSKNTAYLQMNNLKTEDTAVYYCVRHGNFGNSYVSWFAYWGQGTLVTVSSASTKGPSVFPLAPSSKSTSGGTAALGCLVKDYFPEPVTVSWNSGALTSGVHTFPAVLQSSGLYSLSSVVTVPSSSLGTQTYICNVNHKPSNTKVDKKVE

SEQ ID NO: 157 - protein, 478 aa, synthetic construct
ELVVTQEPSLTVSPGGTVTLTCRSSTGAVTTSNYANWVQQKPGQAPRGLIGGTNKRAPGTPARFSGSLLGGKAALTLSGVQPEDEAEYYCALWYPNPWVFGGGTKLTVLRTVAAPSVFIFPPSDEQLKSGTASVVCLLNNFYPREAKVQWKVDNALQSGNSQESVTEQDSKDSTYSLSSTLTLSKADYEKHKVYACEVTHQGLSSPVTKSFNRGECGGGGSEGKSSGSGSESKSTEGKSSGSGSESKSTGGGGSEVQLLESGGGLVQPGGSLKLSCAASGFTFNTYAMNWVRQAPGKGLEWVARIRSKYNNYATYYADSVKDRFTISRDDSKNTAYLQMNNLKTEDTAVYYCVRHGMFGNSYVSWFAYWGQGTLVTVSSASTKGPSVFPLAPSSKSTSGGTAALGCLVKDYFPEPVTVSWNSGALTSGVHTFPAVLQSSGLYSLSSVVTVPSSSLGTQTYICNVNHKPSNTKVDKKVE

SEQ ID NO: 158 - protein, 478 aa, synthetic construct
ELVVTQEPSLTVSPGGTVTLTCRSSTGAVTTSNYANWVQQKPGQAPRGLIGGTNKRAPGTPARFSGSLLGGKAALTLSGVQPEDEAEYYCALWYPNPWVFGGGTKLTVLRTVAAPSVFIFPPSDEQLKSGTASVVCLLNNFYPREAKVQWKVDNALQSGNSQESVTEQDSKDSTYSLSSTLTLSKADYEKHKVYACEVTHQGLSSPVTKSFNRGECGGGGSEGKSSGSGSESKSTEGKSSGSGSESKSTGGGGSEVQLLESGGGLVQPGGSLKLSCAASGFTFNTYAMNWVRQAPGKGLEWVARIRSKYNNYATYYADSVKDRFTISRDDSKNTAYLQMNNLKTEDTAVYYCVRHGNFGNSYVSWFLYWGQGTLVTVSSASTKGPSVFPLAPSSKSTSGGTAALGCLVKDYFPEPVTVSWNSGALTSGVHTFPAVLQSSGLYSLSSVVTVPSSSLGTQTYICNVNHKPSNTKVDKKVE

SEQ ID NO: 159 - protein, 478 aa, synthetic construct
ELVVTQEPSLTVSPGGTVTLTCRSSTGAVTTSNYANWVQQKPGQAPRGLIGGTNKRAPGTPARFSGSLLGGKAALTLSGVQPEDEAEYYCALWYPNDWVFGGGTKLTVLRTVAAPSVFIFPPSDEQLKSGTASVVCLLNNFYPREAKVQWKVDNALQSGNSQESVTEQDSKDSTYSLSSTLTLSKADYEKHKVYACEVTHQGLSSPVTKSFNRGECGGGGSEGKSSGSGSESKSTEGKSSGSGSESKSTGGGGSEVQLLESGGGLVQPGGSLKLSCAASGFTFNTYAMNWVRQAPGKGLEWVARIRSKYNNYATYYADSVKDRFTISRDDSKNTAYLQMNNLKTEDTAVYYCVRHGNFGNSYVSWFAYWGQGTLVTVSSASTKGPSVFPLAPSSKSTSGGTAALGCLVKDYFPEPVTVSWNSGALTSGVHTFPAVLQSSGLYSLSSVVTVPSSSLGTQTYICNVNHKPSNTKVDKKVE

SEQ ID NO: 160 - protein, 478 aa, synthetic construct
ELVVTQEPSLTVSPGGTVTLTCRSSTGAVTTSNYANWVQQKPGQAPRGLIGGTNKRAPGTPARFSGSLLGGKAALTLSGVQPEDEAEYYCALWYSNPWVFGGGTKLTVLRTVAAPSVFIFPPSDEQLKSGTASVVCLLNNFYPREAKVQWKVDNALQSGNSQESVTEQDSKDSTYSLSSTLTLSKADYEKHKVYACEVTHQGLSSPVTKSFNRGECGGGGSEGKSSGSGSESKSTEGKSSGSGSESKSTGGGGSEVQLLESGGGLVQPGGSLKLSCAASGFTFNTYAMNWVRQAPGKGLEWVARIRSKYNNYATYYADSVKDRFTISRDDSKNTAYLQMNNLKTEDTAVYYCVRHGNFGNDYVSWFAYWGQGTLVTVSSASTKGPSVFPLAPSSKSTSGGTAALGCLVKDYFPEPVTVSWNSGALTSGVHTFPAVLQSSGLYSLSSVVTVPSSSLGTQTYICNVNHKPSNTKVDKKVE

SEQ ID NO: 161 - protein, 365 aa, synthetic construct
RTVAAPSVFIFPPSDEQLKSGTASVVCLLNNFYPREAKVQWKVDNALQSGNSQESVTEQDSKDSTYSLSSTLTLSKADYEKHKVYACEVTHQGLSSPVTKSFNRGECGGGGSEGKSSGSGSESKSTEGKSSGSGSESKSTGGGGSQVQLQQSGSELKKPGASVKVSCKASGYTFTNYGMNWVKQAPGQGLKWMGWINTYTGEPTYTDDFKGRFAFSLDTSVSTAYLQISSLKADDTAVYFCARGGFGSSYWYFDVWGQGSLVTVSSASTKGPSVFPLAPSSKSTSGGTAALGCLVKDYFPEPVTVSWNSGALTSGVHTFPAVLQSSGLYSLSSVVTVPSSSLGTQTYICNVNHKPSNTKVDKKVE

SEQ ID NO: 162 - protein, 220 aa, synthetic construct
QVQLQQSGSELKKPGASVKVSCKASGYTFTNYGMNWVKQAPGQGLKWMGWINTYTGEPTYTDDFKGRFAFSLDTSVSTAYLQISSLKADDTAVYFCARGGFGSSYWYFDVWGQGSLVTVSSASTKGPSVFPLAPSSKSTSGGTAALGCLVKDYFPEPVTVSWNSGALTSGVHTFPAVLQSSGLYSLSSVVTVPSSSLGTQTYICNVNHKPSNTKVDKKVE

SEQ ID NO: 163 - protein, 469 aa, synthetic construct
DIQLTQSPSFLSASVGDRVTITCKASQDVGSAVVWYQQKPGKAPKLLIYWASTRHTGVPSRFSGSGSGTEFTLTISSLQPEDFATYFCQQFTSYPTFGQGTKLEIKRTVAAPSVFIFPPSDEQLKSGTASVVCLLNNFYPREAKVQWKVDNALQSGNSQESVTEQDSKDSTYSLSSTLTLSKADYEKHKVYACEVTHQGLSSPVTKSFNRGECGGGGSEGKSSGSGSESKSTEGKSSGSGSESKSTGGGGSQVQLVQSGAEVKKPGASVKVSCKASGYSFTGYYMHWVRQAPGQGLEWIGRINPYNGATTYSQNFKDRATMTVDTSISTAYMELSRLRSDDTAVYYCVPTGMGYFLMDYWGQGTLVTVSSASTKGPSVFPLAPSSKSTSGGTAALGCLVKDYFPEPVTVSWNSGALTSGVHTFPAVLQSSGLYSLSSVVTVPSSSLGTQTYICNVNHKPSNTKVDKKVE

SEQ ID NO: 164 - protein, 218 aa, synthetic construct
QVQLVQSGAEVKKPGASVKVSCKASGYSFTGYYMHWVRQAPGQGLEWIGRINPYNGATTYSQNFKDRATMTVDTSISTAYMELSRLRSDDTAVYYCVPTGMGYFLMDYWGQGTLVTVSSASTKGPSVFPLAPSSKSTSGGTAALGCLVKDYFPEPVTVSWNSGALTSGVHTFPAVLQSSGLYSLSSVVTVPSSSLGTQTYICNVNHKPSNTKVDKKVE

SEQ ID NO: 165 - protein, 231 aa, synthetic construct
PKSCDKTHTCPPCPAPEAAGGPSVFLFPPKPKDTLMISRTPEVTCVVVDVSHEDPEVKFNWYVDGVEVHNAKTKPREEQYNSTYRVVSVLTVLHQDWLNGKEYKCKVSNKALPAPIEKTISKAKGQPREPQVCTLPPSREEMTKNQVSLSCAVKGFYPSDIAVEWESNGQPENNYKTTPPVLDSDGSFFLVSKLTVDKSRWQQGNVFSCSVMHEALHNHYTQKSLSLSPGK

SEQ ID NO: 166 - protein, 231 aa, synthetic construct
PKSCDKTHTCPPCPAPEAAGGPSVFLFPPKPKDTLMISRTPEVTCVVVDVSHEDPEVKFNWYVDGVEVHNAKTKPREEQYNSTYRVVSVLTVLHQDWLNGKEYKCKVSNKALPAPIEKTISKAKGQPREPQVYTLPPCREEMTKNQVSLWCLVKGFYPSDIAVEWESNGQPENNYKTTPPVLDSDGSFFLYSKLTVDKSRWQQGNVFSCSVMHEALHNHYTQKSLSLSPGK